European Patent Application EP 4 434 533 A1, published September 25, 2024. Title: Artificial complex for tethering chromatids or chromosomes. Applicant: Max-Planck-Gesellschaft zur Forderung der Wissenschaften e.V. The sequence listing filed with the application follows.

SEQUENCE LISTING (80 sequences)

SEQ ID NO: 1 - RNA, 285 nt, synthetic construct
  source 1..285: mol_type = other RNA
atggatagtgctacccatattaaattctcaaaacgtgatgaggacggcaaagagttagctggtgcaactatggagttgcgtgattcatctggtaaaactattagtacatggatttcagatggacaagtgaaagatttctacctgtatccaggaaaatatacatttgtcgaaaccgcagcaccagacggttatgaggtagcaactgctattacctttacagttaatgagcaaggtcaggttactgtaaatggcaaagcaactaaaggtgacgctcatattggatcc

SEQ ID NO: 2 - protein, 95 aa, synthetic construct
MDSATHIKFSKRDEDGKELAGATMELRDSSGKTISTWISDGQVKDFYLYPGKYTFVETAAPDGYEVATAITFTVNEQGQVTVNGKATKGDAHIGS

SEQ ID NO: 3 - RNA, 45 nt, synthetic construct
  source 1..45: mol_type = other RNA
ggttccgcccacatcgtgatggtggacgcctacaagccgacgaag

SEQ ID NO: 4 - protein, 15 aa, synthetic construct
GSAHIVMVDAYKPTK

SEQ ID NO: 5 - RNA, 306 nt, synthetic construct
  source 1..306: mol_type = other RNA
atgacaactgaagaagatagtgctacccatattaaattctcaaaacgtgatgaggacggccgtgagttagctggtgcaactatggagttgcgtgattcatctggtaaaactattagtacatggatttcagatggacatgtgaaggatttctacctgtatccaggaaaatatacatttgtcgaaaccgcagcaccagacggttatgaggtagcaactccaattgaatttacagttaatgaggacggtcaggttactgtagatggtgaagcaactgaaggtgacgctcatactggatccagtggtagc

SEQ ID NO: 6 - protein, 102 aa, synthetic construct
MTTEEDSATHIKFSKRDEDGRELAGATMELRDSSGKTISTWISDGHVKDFYLYPGKYTFVETAAPDGYEVATPIEFTVNEDGQVTVDGEATEGDAHTGSSGS

SEQ ID NO: 7 - RNA, 48 nt, synthetic construct
  source 1..48: mol_type = other RNA
agaggagtacctcacatcgtgatggtggacgcctacaagcggtacaag

SEQ ID NO: 8 - protein, 16 aa, synthetic construct
RGVPHIVMVDAYKRYK

SEQ ID NO: 9 - RNA, 2133 nt, synthetic construct
  source 1..2133: mol_type = other RNA
atgcaggtggatctacgcacgctcggctacagtcagcagcagcaagagaagatcaaaccgaaggtgcgttcgacagtggcgcagcaccacgaggcactggtgggccatgggtttacacacgcgcacatcgttgcgctcagccaacacccggcagcgttagggaccgtcgctgtcacgtatcagcacataatcacggcgttgccagaggcgacacacgaagacatcgttggcgtcggcaaacagtggtccggcgcacgcgccctggaggccttgctcacggatgcgggggagttgagaggtccgccgttacagttggacacaggccaacttgtgaagattgcaaaacgtggcggcgtgaccgcaatggaggcagtgcatgcatcgcgcaatgcactgacgggtgcccccctgaacctgaccccggaccaagtggtggctatcgccagcaacggtggcggcaagcaagcgctcgaaacggtgcagcggctgttgccggtgctgtgccaggaccatggcctgaccccggaccaagtggtggctatcgccagcaacaagggcggcaagcaagcgctcgaaacggtgcagcggctgttgccggtgctgtgccaggaccatggcctgactccggaccaagtggtggctatcgccagccacgatggcggcaagcaagcgctcgaaacggtgcagcggctgttgccggtgctgtgccaggaccatggcctgactccggaccaagtggtggctatcgccagccacgatggcggcaagcaagcgctcgaaacggtgcagcggctgttgccggtgctgtgccaggaccatggcctgaccccggaccaagtggtggctatcgccagcaacattggcggcaagcaagcgctcgaaacggtgcagcggctgttgccggtgctgtgccaggaccatggcctgaccccggaccaagtggtggctatcgccagcaacggtggcggcaagcaagcgctcgaaacggtgcagcggctgttgccggtgctgtgccaggaccatggcctgaccccggaccaagtggtggctatcgccagcaacattggcggcaagcaagcgctcgaaacggtgcagcggctgttgccggtgctgtgccaggaccatggcctgaccccggaccaagtggtggctatcgccagcaacggtggcggcaagcaagcgctcgaaacggtgcagcggctgttgccggtgctgtgccaggaccatggcctgaccccggaccaagtggtggctatcgccagcaacggtggcggcaagcaagcgctcgaaacggtgcagcggctgttgccggtgctgtgccaggaccatggcctgactccggaccaagtggtggctatcgccagccacgatggcggcaagcaagcgctcgaaacggtgcagcggctgttgccggtgctgtgccaggaccatggcctgaccccggaccaagtggtggctatcgccagccacgatggcggcaagcaagcgctcgaaacggtgcagcggctgttgccggtgctgtgccaggaccatggcctgaccccggaccaagtggtggctatcgccagcaacattggcggcaagcaagcgctcgaaacggtgcagcggctgttgccggtgctgtgccaggaccatggcctgactccggaccaagtggtggctatcgccagccacgatggcggcaagcaagcgctcgaaacggtgcagcggctgttgccggtgctgtgccaggaccatggcctgaccccggaccaagtggtggctatcgccagcaacaagggcggcaagcaagcgctcgaaacggtgcagcggctgttgccggtgctgtgccaggaccatggcctgaccccggaccaagtggtggctatcgccagcaacggtggcggcaagcaagcgctcgaaagcattgtggcccagctgagccggcctgatccggcgttggccgcgttgaccaacgaccacctcgtcgccttggcctgcctcggcggacgtcctgccatggatgcagtgaaaaagggattgccgcacgcgccggaattgatcagaagagtcaatcgccgtattggcgaacgcacgtcccatcgcgttgcgggatccactggaggcggaggtggctccggcaccgcctcctcc

SEQ ID NO: 10 - protein, 711 aa, synthetic construct
MQVDLRTLGYSQQQQEKIKPKVRSTVAQHHEALVGHGFTHAHIVALSQHPAALGTVAVTYQHIITALPEATHEDIVGVGKQWSGARALEALLTDAGELRGPPLQLDTGQLVKIAKRGGVTAMEAVHASRNALTGAPLNLTPDQVVAIASNGGGKQALETVQRLLPVLCQDHGLTPDQVVAIASNKGGKQALETVQRLLPVLCQDHGLTPDQVVAIASHDGGKQALETVQRLLPVLCQDHGLTPDQVVAIASHDGGKQALETVQRLLPVLCQDHGLTPDQVVAIASNIGGKQALETVQRLLPVLCQDHGLTPDQVVAIASNGGGKQALETVQRLLPVLCQDHGLTPDQVVAIASNIGGKQALETVQRLLPVLCQDHGLTPDQVVAIASNGGGKQALETVQRLLPVLCQDHGLTPDQVVAIASNGGGKQALETVQRLLPVLCQDHGLTPDQVVAIASHDGGKQALETVQRLLPVLCQDHGLTPDQVVAIASHDGGKQALETVQRLLPVLCQDHGLTPDQVVAIASNIGGKQALETVQRLLPVLCQDHGLTPDQVVAIASHDGGKQALETVQRLLPVLCQDHGLTPDQVVAIASNKGGKQALETVQRLLPVLCQDHGLTPDQVVAIASNGGGKQALESIVAQLSRPDPALAALTNDHLVALACLGGRPAMDAVKKGLPHAPELIRRVNRRIGERTSHRVAGSTGGGGGSGTASS

SEQ ID NO: 11 - DNA, 15 bp, synthetic construct
  source 1..15: mol_type = other DNA
tgccatattccacgt

SEQ ID NO: 12 - RNA, 411 nt, Mus musculus
  source 1..411: mol_type = other RNA
acaagtttgtacaaaaaagcaggctccgcggccgcccccttcaccatgctcagacaaaggccacagctggagactgaggagacagtggaggaagagagagcagcagatgaggaagagaggagaaagactgaagctctgagcgagatcgaggttctgagggaggcccaggagcccagtggtcccctcatgctgtcttcagagctctccctagaagcagcagaagatgaaaagtctcgtactagcctcatccccccagaatggtgggcctggtctgaggaggggcagcccgagccccctgcactgcccatgctgcctgaacttcctgaagtgcccatggagatgcccccaaggcctgaactctcttcagaggctaagggtgggcgcgccgacccagctttcttgtacaaagtg

SEQ ID NO: 13 - protein, 137 aa, Mus musculus
TSLYKKAGSAAAPFTMLRQRPQLETEETVEEERAADEEERRKTEALSEIEVLREAQEPSGPLMLSSELSLEAAEDEKSRTSLIPPEWWAWSEEGQPEPPALPMLPELPEVPMEMPPRPELSSEAKGGRADPAFLYKV

SEQ ID NO: 14 - RNA, 24 nt, Mus musculus
  source 1..24: mol_type = other RNA
gagacagtggaggaagagagagca

SEQ ID NO: 15 - protein, 8 aa, Mus musculus
ETVEEERA

SEQ ID NO: 16 - RNA, 21 nt, Mus musculus
  source 1..21: mol_type = other RNA
gagatcgaggttctgagggag

SEQ ID NO: 17 - protein, 7 aa, Mus musculus
EIEVLRE

SEQ ID NO: 18 - RNA, 51 nt, synthetic construct
  source 1..51: mol_type = other RNA
accggtacaagtttgtacaaaaaagcaggctccgcggccgcccccttcacc

SEQ ID NO: 19 - protein, 17 aa, synthetic construct
TGTSLYKKAGSAAAPFT

SEQ ID NO: 20 - RNA, 1137 nt, synthetic construct
  source 1..1137: mol_type = other RNA
accggtatggtgagcaagggcgaggaggataacatggccatcatcaaggagttcatgcgcttcaaggtgcacatggagggctccgtgaacggccacgagttcgagatcgagggcgagggcgagggccgcccctacgagggcacccagaccgccaagctgaaggtgaccaagggtggccccctgcccttcgcctgggacatcctgtcccctcagttcatgtacggctccaaggcctacgtgaagcaccccgccgacatccccgactacttgaagctgtccttccccgagggcttcaagtgggagcgcgtgatgaacttcgaggacggcggcgtggtgaccgtgacccaggactcctccctgcaggacggcgagttcatctacaaggtgaagctgcgcggcaccaacttcccctccgacggccccgtaatgcagaagaagaccatgggctgggaggcctcctccgagcggatgtaccccgaggacggcgccctgaagggcgagatcaagcagaggctgaagctgaaggacggcggccactacgacgctgaggtcaagaccacctacaaggccaagaagcccgtgcagctgcccggcgcctacaacgtcaacatcaagttggacatcacctcccacaacgaggactacaccatcgtggaacagtacgaacgcgccgagggccgccactccaccggcggcatggacgagctgtacaagggtacaagtttgtacaaaaaagcaggctccgcggccgcccccttcaccatgctcagacaaaggccacagctggagactgaggagacagtggaggaagagagagcagcagatgaggaagagaggagaaagactgaagctctgagcgagatcgaggttctgagggaggcccaggagcccagtggtcccctcatgctgtcttcagagctctccctagaagcagcagaagatgaaaagtctcgtactagcctcatccccccagaatggtgggcctggtctgaggaggggcagcccgagccccctgcactgcccatgctgcctgaacttcctgaagtgcccatggagatgcccccaaggcctgaactctcttcagaggctaagggtgggcgcgccgacccagctttcttgtacaaagtggtaagctta

SEQ ID NO: 21 - protein, 379 aa, synthetic construct
TGMVSKGEEDNMAIIKEFMRFKVHMEGSVNGHEFEIEGEGEGRPYEGTQTAKLKVTKGGPLPFAWDILSPQFMYGSKAYVKHPADIPDYLKLSFPEGFKWERVMNFEDGGVVTVTQDSSLQDGEFIYKVKLRGTNFPSDGPVMQKKTMGWEASSERMYPEDGALKGEIKQRLKLKDGGHYDAEVKTTYKAKKPVQLPGAYNVNIKLDITSHNEDYTIVEQYERAEGRHSTGGMDELYKGTSLYKKAGSAAAPFTMLRQRPQLETEETVEEERAADEEERRKTEALSEIEVLREAQEPSGPLMLSSELSLEAAEDEKSRTSLIPPEWWAWSEEGQPEPPALPMLPELPEVPMEMPPRPELSSEAKGGRADPAFLYKVVSL

SEQ ID NO: 22 - RNA, 1866 nt, synthetic construct
  source 1..1866: mol_type = other RNA
accggtatggtgagcaagggcgaggaggataacatggccatcatcaaggagttcatgcgcttcaaggtgcacatggagggctccgtgaacggccacgagttcgagatcgagggcgagggcgagggccgcccctacgagggcacccagaccgccaagctgaaggtgaccaagggtggccccctgcccttcgcctgggacatcctgtcccctcagttcatgtacggctccaaggcctacgtgaagcaccccgccgacatccccgactacttgaagctgtccttccccgagggcttcaagtgggagcgcgtgatgaacttcgaggacggcggcgtggtgaccgtgacccaggactcctccctgcaggacggcgagttcatctacaaggtgaagctgcgcggcaccaacttcccctccgacggccccgtaatgcagaagaagaccatgggctgggaggcctcctccgagcggatgtaccccgaggacggcgccctgaagggcgagatcaagcagaggctgaagctgaaggacggcggccactacgacgctgaggtcaagaccacctacaaggccaagaagcccgtgcagctgcccggcgcctacaacgtcaacatcaagttggacatcacctcccacaacgaggactacaccatcgtggaacagtacgaacgcgccgagggccgccactccaccggcggcatggacgagctgtacaagggtacaagtttgtacaaaaaagcaggctccgcggccgcccccttcaccatgctcagacaaaggccacagctggagactgaggagacagtggaggaagagagagcagcagatgaggaagagaggagaaagactgaagctctgagcgagatcgaggttctgagggaggcccaggagcccagtggtcccctcatgctgtcttcagagctctccctagaagcagcagaagatgaaaagtctcgtactagcctcatccccccagaatggtgggcctggtctgaggaggggcagcccgagccccctgcactgcccatgctgcctgaacttcctgaagtgcccatggagatgcccccaaggcctgaactctcttcagaggctaagggtgggcgcgccgacccagctttcttgtacaaagtggtaagcttcgaattcatggtgagcaagggcgaggagctgttcaccggggtggtgcccatcctggtcgagctggacggcgacgtaaacggccacaagttcagcgtccgcggcgagggcgagggcgatgccaccaacggcaagctgaccctgaagttcatctgcaccaccggcaagctgcccgtgccctggcccaccctcgtgaccaccttcggctacggcgtggcctgcttcagccgctaccccgaccacatgaagcagcacgacttcttcaagtccgccatgcccgaaggctacgtccaggagcgcaccatctctttcaaggacgacggtacctacaagacccgcgccgaggtgaagttcgagggcgacaccctggtgaaccgcatcgagctgaagggcatcgacttcaaggaggacggcaacatcctggggcacaagctggagtacaacttcaacagccacaacgtctatatcacggccgacaagcagaagaacggcatcaaggctaacttcaagatccgccacaacgttgaggacggcagcgtgcagctcgccgaccactaccagcagaacacccccatcggcgacggccccgtgctgctgcccgacaaccactacctgagccatcagtccaagctgagcaaagaccccaacgagaagcgcgatcacatggtcctgctggagttcgtgaccgccgccgggattacacatggcatggacgagctgtacaaggtcgac

SEQ ID NO: 23 - protein, 622 aa, synthetic construct
TGMVSKGEEDNMAIIKEFMRFKVHMEGSVNGHEFEIEGEGEGRPYEGTQTAKLKVTKGGPLPFAWDILSPQFMYGSKAYVKHPADIPDYLKLSFPEGFKWERVMNFEDGGVVTVTQDSSLQDGEFIYKVKLRGTNFPSDGPVMQKKTMGWEASSERMYPEDGALKGEIKQRLKLKDGGHYDAEVKTTYKAKKPVQLPGAYNVNIKLDITSHNEDYTIVEQYERAEGRHSTGGMDELYKGTSLYKKAGSAAAPFTMLRQRPQLETEETVEEERAADEEERRKTEALSEIEVLREAQEPSGPLMLSSELSLEAAEDEKSRTSLIPPEWWAWSEEGQPEPPALPMLPELPEVPMEMPPRPELSSEAKGGRADPAFLYKVVSFEFMVSKGEELFTGVVPILVELDGDVNGHKFSVRGEGEGDATNGKLTLKFICTTGKLPVPWPTLVTTFGYGVACFSRYPDHMKQHDFFKSAMPEGYVQERTISFKDDGTYKTRAEVKFEGDTLVNRIELKGIDFKEDGNILGHKLEYNFNSHNVYITADKQKNGIKANFKIRHNVEDGSVQLADHYQQNTPIGDGPVLLPDNHYLSHQSKLSKDPNEKRDHMVLLEFVTAAGITHGMDELYKVD

SEQ ID NO: 24 - RNA, 2496 nt, synthetic construct
  source 1..2496: mol_type = other RNA
atggtagatttgagaactttgggatattcacagcagcagcaggaaaagatcaagcccaaagtgaggtcgacagtcgcgcagcatcacgaagcgctggtgggtcatgggtttacacatgcccacatcgtagccttgtcgcagcaccctgcagcccttggcacggtcgccgtcaagtaccaggacatgattgcggcgttgccggaagccacacatgaggcgatcgtcggtgtggggaaacagtggagcggagcccgagcgcttgaggccctgttgacggtcgcgggagagctgagagggcctccccttcagctggacacgggccagttgctgaagatcgcgaagcggggaggagtcacggcggtcgaggcggtgcacgcgtggcgcaatgcgctcacgggagcacccctcaacctgaccccagagcaggtcgtggcaattgcgagccatgacgggggaaagcaggcactcgaaaccgtccagaggttgctgcctgtgctgtgccaagcgcacggacttacgccagagcaggtcgtggcaattgcgagccatgacgggggaaagcaggcactcgaaaccgtccagaggttgctgcctgtgctgtgccaagcgcacggactaaccccagagcaggtcgtggcaattgcgagcaacatcgggggaaagcaggcactcgaaaccgtccagaggttgctgcctgtgctgtgccaagcgcacgggttgaccccagagcaggtcgtggcaattgcgagcaacggagggggaaagcaggcactcgaaaccgtccagaggttgctgcctgtgctgtgccaagcgcacgggttgaccccagagcaggtcgtggcaattgcgagcaacggagggggaaagcaggcactcgaaaccgtccagaggttgctgcctgtgctgtgccaagcgcacggactgacaccagagcaggtcgtggcaattgcgagccatgacgggggaaagcaggcactcgaaaccgtccagaggttgctgcctgtgctgtgccaagcgcacggacttacacccgaacaagtcgtggcaattgcgagccatgacgggggaaagcaggcactcgaaaccgtccagaggttgctgcctgtgctgtgccaagcgcacggactaaccccagagcaggtcgtggcaattgcgagcaacatcgggggaaagcaggcactcgaaaccgtccagaggttgctgcctgtgctgtgccaagcgcacgggttgaccccagagcaggtcgtggcaattgcgagcaacggagggggaaagcaggcactcgaaaccgtccagaggttgctgcctgtgctgtgccaagcgcacgggttgaccccagagcaggtcgtggcaattgcgagcaacggagggggaaagcaggcactcgaaaccgtccagaggttgctgcctgtgctgtgccaagcgcacggactgacaccagagcaggtcgtggcaattgcgagccatgacgggggaaagcaggcactcgaaaccgtccagaggttgctgcctgtgctgtgccaagcgcacggacttacacccgaacaagtcgtggcaattgcgagccatgacgggggaaagcaggcactcgaaaccgtccagaggttgctgcctgtgctgtgccaagcgcacggcctcaccccagagcaggtcgtggcaattgcgagcaacatcgggggaaagcaggcactcgaaaccgtccagaggttgctgcctgtgctgtgccaagcgcacggacttacgccagagcaggtcgtggcaattgcgagcaacggagggggaaagcaggcactcgaaaccgtccagaggttgctgcctgtgctgtgccaagcgcacggactaaccccagagcaggtcgtggcaattgcgagcaacggagggggaaagcaggcactcgaaaccgtccagaggttgctgcctgtgctgtgccaagcgcacgggttgaccccagagcaggtcgtggcaattgcgagccatgacgggggaaagcaggcactcgaaaccgtccagaggttgctgcctgtgctgtgccaagcgcacggcctgaccccagagcaggtcgtggcaattgcgagccatgacgggggaaagcaggcactcgaaaccgtccagaggttgctgcctgtgctgtgccaagcgcacggactgacaccagagcaggtcgtggcaattgcgagcaacatcgggggaaagcaggcactcgaaaccgtccagaggttgctgcctgtgctgtgccaagcgcacggactcacgcctgagcaggtagtggctattgcatccaacggagggggcagacccgcactggagtcaatcgtggcccagctttcgaggccggaccccgcgctggccgcactcactaatgatcatcttgtagcgctggcctgcctcggcggacgacccgccttggatgcggtgaagaaggggctcccgcacgcgcctgcattgattaagcggaccaacagaaggattcccgagaggacatcacatcgagtggca

SEQ ID NO: 25 - protein, 832 aa, synthetic construct
MVDLRTLGYSQQQQEKIKPKVRSTVAQHHEALVGHGFTHAHIVALSQHPAALGTVAVKYQDMIAALPEATHEAIVGVGKQWSGARALEALLTVAGELRGPPLQLDTGQLLKIAKRGGVTAVEAVHAWRNALTGAPLNLTPEQVVAIASHDGGKQALETVQRLLPVLCQAHGLTPEQVVAIASHDGGKQALETVQRLLPVLCQAHGLTPEQVVAIASNIGGKQALETVQRLLPVLCQAHGLTPEQVVAIASNGGGKQALETVQRLLPVLCQAHGLTPEQVVAIASNGGGKQALETVQRLLPVLCQAHGLTPEQVVAIASHDGGKQALETVQRLLPVLCQAHGLTPEQVVAIASHDGGKQALETVQRLLPVLCQAHGLTPEQVVAIASNIGGKQALETVQRLLPVLCQAHGLTPEQVVAIASNGGGKQALETVQRLLPVLCQAHGLTPEQVVAIASNGGGKQALETVQRLLPVLCQAHGLTPEQVVAIASHDGGKQALETVQRLLPVLCQAHGLTPEQVVAIASHDGGKQALETVQRLLPVLCQAHGLTPEQVVAIASNIGGKQALETVQRLLPVLCQAHGLTPEQVVAIASNGGGKQALETVQRLLPVLCQAHGLTPEQVVAIASNGGGKQALETVQRLLPVLCQAHGLTPEQVVAIASHDGGKQALETVQRLLPVLCQAHGLTPEQVVAIASHDGGKQALETVQRLLPVLCQAHGLTPEQVVAIASNIGGKQALETVQRLLPVLCQAHGLTPEQVVAIASNGGGRPALESIVAQLSRPDPALAALTNDHLVALACLGGRPALDAVKKGLPHAPALIKRTNRRIPERTSHRVA

SEQ ID NO: 26 - DNA, 19 bp, synthetic construct
  source 1..19: mol_type = other DNA
ccattccattccattccat

SEQ ID NO: 27 - RNA, 333 nt, Homo sapiens
  source 1..333: mol_type = other RNA
cattgtgcccagccacccccaaaagccctcaggcgagagctgcctgaggaggcagccgctgaggaggaaaggagaaagattgaagttccaagtgagattgaggtcccgagggaggccctggagcccagtgttccccttatggtgtctttagagatctccctagaggcagctgaagaggagaagtcccgcatcagcctcatcccaccagaagaacggtgggcctggcctgaggtggaggcgccagaagctcctgcattgcccgtggtgcctgaactccctgaggtgcccatggagatgcctttggtgctgcccccagagctcgagctgctcatc

SEQ ID NO: 28 - protein, 111 aa, Homo sapiens
HCAQPPPKALRRELPEEAAAEEERRKIEVPSEIEVPREALEPSVPLMVSLEISLEAAEEEKSRISLIPPEERWAWPEVEAPEAPALPVVPELPEVPMEMPLVLPPELELLI

SEQ ID NO: 29 - protein, 12 aa, Homo sapiens
GAGGAGGAAAGG

SEQ ID NO: 30 - protein, 4 aa, Homo sapiens
EEER

SEQ ID NO: 31 - RNA, 12 nt, Homo sapiens
  source 1..12: mol_type = other RNA
gaggtcccgagg

SEQ ID NO: 32 - protein, 4 aa, Homo sapiens
EVPR

SEQ ID NO: 33 - RNA, 51 nt, synthetic construct; identical to SEQ ID NO: 18
  source 1..51: mol_type = other RNA

SEQ ID NO: 34 - protein, 17 aa, synthetic construct
TGTSLYKKAGSAAAPFT

SEQ ID NO: 35 - RNA, 1053 nt, synthetic construct
  source 1..1053: mol_type = other RNA
aaagtggtccattgtgcccagccacccccaaaagccctcaggcgagagctgcctgaggaggcagccgctgaggaggaaaggagaaagattgaagttccaagtgagattgaggtcccgagggaggccctggagcccagtgttccccttatggtgtctttagagatctccctagaggcagctgaagaggagaagtcccgcatcagcctcatcccaccagaagaacggtgggcctggcctgaggtggaggcgccagaagctcctgcattgcccgtggtgcctgaactccctgaggtgcccatggagatgcctttggtgctgcccccagagctcgagctgctcagaatggtgagcaagggcgaggaggataacatggccatcatcaaggagttcatgcgcttcaaggtgcacatggagggctccgtgaacggccacgagttcgagatcgagggcgagggcgagggccgcccctacgagggcacccagaccgccaagctgaaggtgaccaagggtggccccctgcccttcgcctgggacatcctgtcccctcagttcatgtacggctccaaggcctacgtgaagcaccccgccgacatccccgactacttgaagctgtccttccccgagggcttcaagtgggagcgcgtgatgaacttcgaggacggcggcgtggtgaccgtgacccaggactcctccctgcaggacggcgagttcatctacaaggtgaagctgcgcggcaccaacttcccctccgacggccccgtaatgcagaagaagaccatgggctgggaggcctcctccgagcggatgtaccccgaggacggcgccctgaagggcgagatcaagcagaggctgaagctgaaggacggcggccactacgacgctgaggtcaagaccacctacaaggccaagaagcccgtgcagctgcccggcgcctacaacgtcaacatcaagttggacatcacctcccacaacgaggactacaccatcgtggaacagtacgaacgcgccgagggccgccactccaccggcggcatggacgagctgtacaagaaa

SEQ ID NO: 36 - protein, 351 aa, synthetic construct
KVVHCAQPPPKALRRELPEEAAAEEERRKIEVPSEIEVPREALEPSVPLMVSLEISLEAAEEEKSRISLIPPEERWAWPEVEAPEAPALPVVPELPEVPMEMPLVLPPELELLRMVSKGEEDNMAIIKEFMRFKVHMEGSVNGHEFEIEGEGEGRPYEGTQTAKLKVTKGGPLPFAWDILSPQFMYGSKAYVKHPADIPDYLKLSFPEGFKWERVMNFEDGGVVTVTQDSSLQDGEFIYKVKLRGTNFPSDGPVMQKKTMGWEASSERMYPEDGALKGEIKQRLKLKDGGHYDAEVKTTYKAKKPVQLPGAYNVNIKLDITSHNEDYTIVEQYERAEGRHSTGGMDELYKK

SEQ ID NO: 37 - RNA, 1113 nt, synthetic construct
  source 1..1113: mol_type = other RNA
aagggtgggcgcgccgacccagctttcttgtacaaagtggtctcgagctcacattgtgcccagccacccccaaaagccctcaggcgagagctgcctgaggaggcagccgctgaggaggaaaggagaaagattgaagttccaagtgagattgaggtcccgagggaggccctggagcccagtgttccccttatggtgtctttagagatctccctagaggcagctgaagaggagaagtcccgcatcagcctcatcccaccagaagaacggtgggcctggcctgaggtggaggcgccagaagctcctgcattgcccgtggtgcctgaactccctgaggtgcccatggagatgcctttggtgctgcccccagagctcgagctgctcatcgaattcatggtgagcaagggcgaggagctgttcaccggggtggtgcccatcctggtcgagctggacggcgacgtaaacgaccacaagttcagcgtccgcggcgagggcgagggcgatgccaccaacggcaagctgaccctgaagttcatctgcaccaccggcaagctgcccgtgccctggcccaccctcgtgaccaccttcggctacggcgtggcctgcttcagccgctaccccgaccacatgaagcagcacgacttcttcaagtccgccatgcccgaaggctacgtccaggagcgcaccatctctttcaaggacgacggtacctacaagacccgcgccgaggtgaagttcgagggcgacaccctggtgaaccgcatcgagctgaagggcatcgacttcaaggaggacggcaacatcctggggcacaagctggagtacaacttcaacagccacaacgtctatatcacggccgacaagcagaagaacggcatcaaggctaacttcaagatccgccacaacgttgaggacggcagcgtgcagctcgccgaccactaccagcagaacacccccatcggcgacggccccgtgctgctgcccgacaaccactacctgagccatcagtccaagctgagcaaagaccccaacgagaagcgcgatcacatggtcctgctggagttcgtgaccgccgccgggattacacatggcatggacgagctgtacaaggtcgac

SEQ ID NO: 38 - protein, 371 aa, synthetic construct
KGGRADPAFLYKVVSSSHCAQPPPKALRRELPEEAAAEEERRKIEVPSEIEVPREALEPSVPLMVSLEISLEAAEEEKSRISLIPPEERWAWPEVEAPEAPALPVVPELPEVPMEMPLVLPPELELLIEFMVSKGEELFTGVVPILVELDGDVNDHKFSVRGEGEGDATNGKLTLKFICTTGKLPVPWPTLVTTFGYGVACFSRYPDHMKQHDFFKSAMPEGYVQERTISFKDDGTYKTRAEVKFEGDTLVNRIELKGIDFKEDGNILGHKLEYNFNSHNVYITADKQKNGIKANFKIRHNVEDGSVQLADHYQQNTPIGDGPVLLPDNHYLSHQSKLSKDPNEKRDHMVLLEFVTAAGITHGMDELYKVD

SEQ ID NO: 39 - RNA, 447 nt, synthetic construct
  source 1..447: mol_type = other RNA
atggagtttctggcaaccacactggaacggatcgagaaaaatttcgtgattactgatccgagactgcctgacaacccaatcatttttgcgagcgattccttcctgcagctgacagaatattctcgggaagagatcctggggcgcaattgccgttttctgcagggacccgagacagaccgtgccactgttcggaaaatcagagatgctattgacaaccagactgaagtgaccgttcagctgatcaattataccaagagcggcaagaagttctggaacgtgttccacctgcagccgatgcgcgattataagggcgacgtccagtacttcattggcgtgcagctggatggcaccgaacgtcttcatggcgccgctgagcgtgaggcggtcatgctgatcaaaaagacagccgcccacatcgtgatggtggacgcctacaagccgacgaag

SEQ ID NO: 40 - protein, 149 aa, synthetic construct
MEFLATTLERIEKNFVITDPRLPDNPIIFASDSFLQLTEYSREEILGRNCRFLQGPETDRATVRKIRDAIDNQTEVTVQLINYTKSGKKFWNVFHLQPMRDYKGDVQYFIGVQLDGTERLHGAAEREAVMLIKKTAAHIVMVDAYKPTK

SEQ ID NO: 41 - RNA, 717 nt, synthetic construct
  source 1..717: mol_type = other RNA
atggtgagcaagggcgaggagctgttcaccggggtggtgcccatcctggtcgagctggacggcgacgtaaacggccacaagttcagcgtccgcggcgagggcgagggcgatgccaccaacggcaagctgaccctgaagttcatctgcaccaccggcaagctgcccgtgccctggcccaccctcgtgaccaccttcggctacggcgtggcctgcttcagccgctaccccgaccacatgaagcagcacgacttcttcaagtccgccatgcccgaaggctacgtccaggagcgcaccatctctttcaaggacgacggtacctacaagacccgcgccgaggtgaagttcgagggcgacaccctggtgaaccgcatcgagctgaagggcatcgacttcaaggaggacggcaacatcctggggcacaagctggagtacaacttcaacagccacaacgtctatatcacggccgacaagcagaagaacggcatcaaggctaacttcaagatccgccacaacgttgaggacggcagcgtgcagctcgccgaccactaccagcagaacacccccatcggcgacggccccgtgctgctgcccgacaaccactacctgagccatcagtccaagctgagcaaagaccccaacgagaagcgcgatcacatggtcctgctggagttcgtgaccgccgccgggattacacatggcatggacgagctgtacaag

SEQ ID NO: 42 - protein, 239 aa, synthetic construct
MVSKGEELFTGVVPILVELDGDVNGHKFSVRGEGEGDATNGKLTLKFICTTGKLPVPWPTLVTTFGYGVACFSRYPDHMKQHDFFKSAMPEGYVQERTISFKDDGTYKTRAEVKFEGDTLVNRIELKGIDFKEDGNILGHKLEYNFNSHNVYITADKQKNGIKANFKIRHNVEDGSVQLADHYQQNTPIGDGPVLLPDNHYLSHQSKLSKDPNEKRDHMVLLEFVTAAGITHGMDELYK

SEQ ID NO: 43 - RNA, 708 nt, synthetic construct
  source 1..708: mol_type = other RNA
atggtgagcaagggcgaggaggataacatggccatcatcaaggagttcatgcgcttcaaggtgcacatggagggctccgtgaacggccacgagttcgagatcgagggcgagggcgagggccgcccctacgagggcacccagaccgccaagctgaaggtgaccaagggtggccccctgcccttcgcctgggacatcctgtcccctcagttcatgtacggctccaaggcctacgtgaagcaccccgccgacatccccgactacttgaagctgtccttccccgagggcttcaagtgggagcgcgtgatgaacttcgaggacggcggcgtggtgaccgtgacccaggactcctccctgcaggacggcgagttcatctacaaggtgaagctgcgcggcaccaacttcccctccgacggccccgtaatgcagaagaagaccatgggctgggaggcctcctccgagcggatgtaccccgaggacggcgccctgaagggcgagatcaagcagaggctgaagctgaaggacggcggccactacgacgctgaggtcaagaccacctacaaggccaagaagcccgtgcagctgcccggcgcctacaacgtcaacatcaagttggacatcacctcccacaacgaggactacaccatcgtggaacagtacgaacgcgccgagggccgccactccaccggcggcatggacgagctgtacaag

SEQ ID NO: 44 - protein, 236 aa, synthetic construct
MVSKGEEDNMAIIKEFMRFKVHMEGSVNGHEFEIEGEGEGRPYEGTQTAKLKVTKGGPLPFAWDILSPQFMYGSKAYVKHPADIPDYLKLSFPEGFKWERVMNFEDGGVVTVTQDSSLQDGEFIYKVKLRGTNFPSDGPVMQKKTMGWEASSERMYPEDGALKGEIKQRLKLKDGGHYDAEVKTTYKAKKPVQLPGAYNVNIKLDITSHNEDYTIVEQYERAEGRHSTGGMDELYK

SEQ ID NO: 45 - RNA, 303 nt, Mus musculus
  source 1..303: mol_type = other RNA
atggctactcttatctttgttgataaggataatgaagaacccggccgccgtttggcatctaaggatgggttgaagctgggcactggtgtcaaggccttagatgggaaattgcaggtttcaacgcctcgagtcggcaaagtgttcaatgctccagccgtgcctaaagccagcagaaaggctttggggacagtcaacagagttgccgaaaagcctatgaagactggcaaacccctccaaccaaaacagccgaccttgactgggaaaaagatcaccgagaagtctactaagacacaaagttctgtt

SEQ ID NO: 46 - protein, 101 aa, Mus musculus
MATLIFVDKDNEEPGRRLASKDGLKLGTGVKALDGKLQVSTPRVGKVFNAPAVPKASRKALGTVNRVAEKPMKTGKPLQPKQPTLTGKKITEKSTKTQSSV

SEQ ID NO: 47 - RNA, 237 nt, Mus musculus
  source 1..237: mol_type = other RNA
atggcgctcagggtcactaggaacacgaaaattaacgcagaaaataaggccaaggtcagtatggcaggcgccaagcgtgtgcctgtgacagttactgctgcttccaagcccgggctgagaccgagaactgctcttggagacattggtaataaagtcagcgaagagctacaggcaagagtgcctctgaaaagggaagcaaaaacgctaggtactggaaaaggtactgttaaagcccta

SEQ ID NO: 48 - protein, 79 aa, Mus musculus
MALRVTRNTKINAENKAKVSMAGAKRVPVTVTAASKPGLRPRTALGDIGNKVSEELQARVPLKREAKTLGTGKGTVKAL

SEQ ID NO: 49 - RNA, 52 nt, synthetic construct
  source 1..52: mol_type = other RNA
gacaccgaggacgtggtgtgctgcagcatgagctacacctggaccggcaaga

SEQ ID NO: 50 - protein, 17 aa, synthetic construct
DTEDVVCCSMSYTWTGK

SEQ ID NO: 51 - RNA, 3426 nt, synthetic construct
  source 1..3426: mol_type = other RNA
gcgaattaattcgagctcggtacccagcttgcttgttctttttgcagaagctcagaataaacgctcaactttggcagatcaattccccggtgctagcatgggttccgcccacatcgtgatggtggacgcctacaagccgacgaagaccggtacaagtttgtacaaaaaagcaggctccgcggccgcccccttcaccatgcaggtggatctacgcacgctcggctacagtcagcagcagcaagagaagatcaaaccgaaggtgcgttcgacagtggcgcagcaccacgaggcactggtgggccatgggtttacacacgcgcacatcgttgcgctcagccaacacccggcagcgttagggaccgtcgctgtcacgtatcagcacataatcacggcgttgccagaggcgacacacgaagacatcgttggcgtcggcaaacagtggtccggcgcacgcgccctggaggccttgctcacggatgcgggggagttgagaggtccgccgttacagttggacacaggccaacttgtgaagattgcaaaacgtggcggcgtgaccgcaatggaggcagtgcatgcatcgcgcaatgcactgacgggtgcccccctgaacctgaccccggaccaagtggtggctatcgccagcaacggtggcggcaagcaagcgctcgaaacggtgcagcggctgttgccggtgctgtgccaggaccatggcctgaccccggaccaagtggtggctatcgccagcaacaagggcggcaagcaagcgctcgaaacggtgcagcggctgttgccggtgctgtgccaggaccatggcctgactccggaccaagtggtggctatcgccagccacgatggcggcaagcaagcgctcgaaacggtgcagcggctgttgccggtgctgtgccaggaccatggcctgactccggaccaagtggtggctatcgccagccacgatggcggcaagcaagcgctcgaaacggtgcagcggctgttgccggtgctgtgccaggaccatggcctgaccccggaccaagtggtggctatcgccagcaacattggcggcaagcaagcgctcgaaacggtgcagcggctgttgccggtgctgtgccaggaccatggcctgaccccggaccaagtggtggctatcgccagcaacggtggcggcaagcaagcgctcgaaacggtgcagcggctgttgccggtgctgtgccaggaccatggcctgaccccggaccaagtggtggctatcgccagcaacattggcggcaagcaagcgctcgaaacggtgcagcggctgttgccggtgctgtgccaggaccatggcctgaccccggaccaagtggtggctatcgccagcaacggtggcggcaagcaagcgctcgaaacggtgcagcggctgttgccggtgctgtgccaggaccatggcctgaccccggaccaagtggtggctatcgccagcaacggtggcggcaagcaagcgctcgaaacggtgcagcggctgttgccggtgctgtgccaggaccatggcctgactccggaccaagtggtggctatcgccagccacgatggcggcaagcaagcgctcgaaacggtgcagcggctgttgccggtgctgtgccaggaccatggcctgaccccggaccaagtggtggctatcgccagccacgatggcggcaagcaagcgctcgaaacggtgcagcggctgttgccggtgctgtgccaggaccatggcctgaccccggaccaagtggtggctatcgccagcaacattggcggcaagcaagcgctcgaaacggtgcagcggctgttgccggtgctgtgccaggaccatggcctgactccggaccaagtggtggctatcgccagccacgatggcggcaagcaagcgctcgaaacggtgcagcggctgttgccggtgctgtgccaggaccatggcctgaccccggaccaagtggtggctatcgccagcaacaagggcggcaagcaagcgctcgaaacggtgcagcggctgttgccggtgctgtgccaggaccatggcctgaccccggaccaagtggtggctatcgccagcaacggtggcggcaagcaagcgctcgaaagcattgtggcccagctgagccggcctgatccggcgttggccgcgttgaccaacgaccacctcgtcgccttggcctgcctcggcggacgtcctgccatggatgcagtgaaaaagggattgccgcacgcgccggaattgatcagaagagtcaatcgccgtattggcgaacgcacgtcccatcgcgttgcgggatccactggaggcggaggtggctccggcaccgcctcctccaagggtgggcgcgccgacccagctttcttgtacaaagtggtctcgagaatggtgagcaagggcgaggaggataacatggccatcatcaaggagttcatgcgcttcaaggtgcacatggagggctccgtgaacggccacgagttcgagatcgagggcgagggcgagggccgcccctacgagggcacccagaccgccaagctgaaggtgaccaagggtggccccctgcccttcgcctgggacatcctgtcccctcagttcatgtacggctccaaggcctacgtgaagcaccccgccgacatccccgactacttgaagctgtccttccccgagggcttcaagtgggagcgcgtgatgaacttcgaggacggcggcgtggtgaccgtgacccaggactcctccctgcaggacggcgagttcatctacaaggtgaagctgcgcggcaccaacttcccctccgacggccccgtaatgcagaagaagaccatgggctgggaggcctcctccgagcggatgtaccccgaggacggcgccctgaagggcgagatcaagcagaggctgaagctgaaggacggcggccactacgacgctgaggtcaagaccacctacaaggccaagaagcccgtgcagctgcccggcgcctacaacgtcaacatcaagttggacatcacctcccacaacgaggactacaccatcgtggaacagtacgaacgcgccgagggccgccactccaccggcggcatggacgagctgtacaagaaaagcttaggttccgcccatatagttatggtggacgcctataaacccactaagagtcgacggcccgggatcctgtacaagtaaagcggccgctctagataaatgatagcttgatctggttaccactaaaccagcctcaagaacacccgaatggagtctctaagctacataataccaacttacactttacaaaatgttgtcccccaaaatgtagccattcgtatctgctcctaataaaaagaaagtttcttcacattctaaaaaaaaaaaaaaaaaaaaaaaaaaaaaaaaaaccccccccccccccccctgcaggcgcgccgccggcgatttaaattaat

SEQ ID NO: 52 - protein, 1023 aa, synthetic construct
MGSAHIVMVDAYKPTKTGTSLYKKAGSAAAPFTMQVDLRTLGYSQQQQEKIKPKVRSTVAQHHEALVGHGFTHAHIVALSQHPAALGTVAVTYQHIITALPEATHEDIVGVGKQWSGARALEALLTDAGELRGPPLQLDTGQLVKIAKRGGVTAMEAVHASRNALTGAPLNLTPDQVVAIASNGGGKQALETVQRLLPVLCQDHGLTPDQVVAIASNKGGKQALETVQRLLPVLCQDHGLTPDQVVAIASHDGGKQALETVQRLLPVLCQDHGLTPDQVVAIASHDGGKQALETVQRLLPVLCQDHGLTPDQVVAIASNIGGKQALETVQRLLPVLCQDHGLTPDQVVAIASNGGGKQALETVQRLLPVLCQDHGLTPDQVVAIASNIGGKQALETVQRLLPVLCQDHGLTPDQVVAIASNGGGKQALETVQRLLPVLCQDHGLTPDQVVAIASNGGGKQALETVQRLLPVLCQDHGLTPDQVVAIASHDGGKQALETVQRLLPVLCQDHGLTPDQVVAIASHDGGKQALETVQRLLPVLCQDHGLTPDQVVAIASNIGGKQALETVQRLLPVLCQDHGLTPDQVVAIASHDGGKQALETVQRLLPVLCQDHGLTPDQVVAIASNKGGKQALETVQRLLPVLCQDHGLTPDQVVAIASNGGGKQALESIVAQLSRPDPALAALTNDHLVALACLGGRPAMDAVKKGLPHAPELIRRVNRRIGERTSHRVAGSTGGGGGSGTASSKGGRADPAFLYKVVSRMVSKGEEDNMAIIKEFMRFKVHMEGSVNGHEFEIEGEGEGRPYEGTQTAKLKVTKGGPLPFAWDILSPQFMYGSKAYVKHPADIPDYLKLSFPEGFKWERVMNFEDGGVVTVTQDSSLQDGEFIYKVKLRGTNFPSDGPVMQKKTMGWEASSERMYPEDGALKGEIKQRLKLKDGGHYDAEVKTTYKAKKPVQLPGAYNVNIKLDITSHNEDYTIVEQYERAEGRHSTGGMDELYKKSLGSAHIVMVDAYKPTKSRRPGILYK

SEQ ID NO: 53 - RNA, 3896 nt, synthetic construct
  source 1..3896: mol_type = other RNA
gcgaattaattcgagctcggtacccagcttgcttgttctttttgcagaagctcagaataaacgctcaactttggcagatcaattccccggtgctagcatggatagtgctacccatattaaattctcaaaacgtgatgaggacggcaaagagttagctggtgcaactatggagttgcgtgattcatctggtaaaactattagtacatggatttcagatggacaagtgaaagatttctacctgtatccaggaaaatatacatttgtcgaaaccgcagcaccagacggttatgaggtagcaactgctattacctttacagttaatgagcaaggtcaggttactgtaaatggcaaagcaactaaaggtgacgctcatattggatccaccggtacaagtttgtacaaaaaagcaggctccgcggccgcccccttcaccatgcaggtggatctacgcacgctcggctacagtcagcagcagcaagagaagatcaaaccgaaggtgcgttcgacagtggcgcagcaccacgaggcactggtgggccatgggtttacacacgcgcacatcgttgcgctcagccaacacccggcagcgttagggaccgtcgctgtcacgtatcagcacataatcacggcgttgccagaggcgacacacgaagacatcgttggcgtcggcaaacagtggtccggcgcacgcgccctggaggccttgctcacggatgcgggggagttgagaggtccgccgttacagttggacacaggccaacttgtgaagattgcaaaacgtggcggcgtgaccgcaatggaggcagtgcatgcatcgcgcaatgcactgacgggtgcccccctgaacctgaccccggaccaagtggtggctatcgccagcaacggtggcggcaagcaagcgctcgaaacggtgcagcggctgttgccggtgctgtgccaggaccatggcctgaccccggaccaagtggtggctatcgccagcaacaagggcggcaagcaagcgctcgaaacggtgcagcggctgttgccggtgctgtgccaggaccatggcctgactccggaccaagtggtggctatcgccagccacgatggcggcaagcaagcgctcgaaacggtgcagcggctgttgccggtgctgtgccaggaccatggcctgactccggaccaagtggtggctatcgccagccacgatggcggcaagcaagcgctcgaaacggtgcagcggctgttgccggtgctgtgccaggaccatggcctgaccccggaccaagtggtggctatcgccagcaacattggcggcaagcaagcgctcgaaacggtgcagcggctgttgccggtgctgtgccaggaccatggcctgaccccggaccaagtggtggctatcgccagcaacggtggcggcaagcaagcgctcgaaacggtgcagcggctgttgccggtgctgtgccaggaccatggcctgaccccggaccaagtggtggctatcgccagcaacattggcggcaagcaagcgctcgaaacggtgcagcggctgttgccggtgctgtgccaggaccatggcctgaccccggaccaagtggtggctatcgccagcaacggtggcggcaagcaagcgctcgaaacggtgcagcggctgttgccggtgctgtgccaggaccatggcctgaccccggaccaagtggtggctatcgccagcaacggtggcggcaagcaagcgctcgaaacggtgcagcggctgttgccggtgctgtgccaggaccatggcctgactccggaccaagtggtggctatcgccagccacgatggcggcaagcaagcgctcgaaacggtgcagcggctgttgccggtgctgtgccaggaccatggcctgaccccggaccaagtggtggctatcgccagccacgatggcggcaagcaagcgctcgaaacggtgcagcggctgttgccggtgctgtgccaggaccatggcctgaccccggaccaagtggtggctatcgccagcaacattggcggcaagcaagcgctcgaaacggtgcagcggctgttgccggtgctgtgccaggaccatggcctgactccggaccaagtggtggctatcgccagccacgatggcggcaagcaagcgctcgaaacggtgcagcggctgttgccggtgctgtgccaggaccatggcctgaccccggaccaagtggtggctatcgccagcaacaagggcggcaagcaagcgctcgaaacggtgcagcggctgttgccggtgctgtgccaggaccatggcctgaccccggaccaagtggtggctatcgccagcaacggtggcggcaagcaagcgctcgaaagcattgtggcccagctgagccggcctgatccggcgttggccgcgttgaccaacgaccacctcgtcgccttggcctgcctcggcggacgtcctgccatggatgcagtgaaaaagggattgccgcacgcgccggaattgatcagaagagtcaatcgccgtattggcgaacgcacgtcccatcgcgttgcgggatccactggaggcggaggtggctccggcaccgcctcctccaagggtgggcgcgccgacccagctttcttgtacaaagtggtctcgagctcaagcttcgaattcatggtgagcaagggcgaggagctgttcaccggggtggtgcccatcctggtcgagctggacggcgacgtaaacgaccacaagttcagcgtccgcggcgagggcgagggcgatgccaccaacggcaagctgaccctgaagttcatctgcaccaccggcaagctgcccgtgccctggcccaccctcgtgaccaccttcggctacggcgtggcctgcttcagccgctaccccgaccacatgaagcagcacgacttcttcaagtccgccatgcccgaaggctacgtccaggagcgcaccatctctttcaaggacgacggtacctacaagacccgcgccgaggtgaagttcgagggcgacaccctggtgaaccgcatcgagctgaagggcatcgacttcaaggaggacggcaacatcctggggcacaagctggagtacaacttcaacagccacaacgtctatatcacggccgacaagcagaagaacggcatcaaggctaacttcaagatccgccacaacgttgaggacggcagcgtgcagctcgccgaccactaccagcagaacacccccatcggcgacggccccgtgctgctgcccgacaaccactacctgagccatcagtccaagctgagcaaagaccccaacgagaagcgcgatcacatggtcctgctggagttcgtgaccgccgccgggattacacatggcatggacgagctgtacaaggtcgacatggatagtgctacccatattaaattctcaaaacgtgatgaggacggcaaagagttagctggtgcaactatggagttgcgtgattcatctggtaaaactattagtacatggatttcagatggacaagtgaaagatttctacctgtatccaggaaaatatacatttgtcgaaaccgcagcaccagacggttatgaggtagcaactgctattacctttacagttaatgagcaaggtcaggttactgtaaatggcaaagcaactaaaggtgacgctcatattggatcctaagcggccgctctagataaatgatagcttgatctggttaccactaaaccagcctcaagaacacccgaatggagtctctaagctacataataccaacttacactttacaaaatgttgtcccccaaaatgtagccattcgtatctgctcctaataaaaagaaagtttcttcacattctaaaaaaaaaaaaaaaaaaaaaaaaaaaaaaaaaaccccccccccccccccctgcaggcgcgccgccggcgatttaaattaat

SEQ ID NO: 54 - protein, 1180 aa, synthetic construct
MDSATHIKFSKRDEDGKELAGATMELRDSSGKTISTWISDGQVKDFYLYPGKYTFVETAAPDGYEVATAITFTVNEQGQVTVNGKATKGDAHIGSTGTSLYKKAGSAAAPFTMQVDLRTLGYSQQQQEKIKPKVRSTVAQHHEALVGHGFTHAHIVALSQHPAALGTVAVTYQHIITALPEATHEDIVGVGKQWSGARALEALLTDAGELRGPPLQLDTGQLVKIAKRGGVTAMEAVHASRNALTGAPLNLTPDQVVAIASNGGGKQALETVQRLLPVLCQDHGLTPDQVVAIASNKGGKQALETVQRLLPVLCQDHGLTPDQVVAIASHDGGKQALETVQRLLPVLCQDHGLTPDQVVAIASHDGGKQALETVQRLLPVLCQDHGLTPDQVVAIASNIGGKQALETVQRLLPVLCQDHGLTPDQVVAIASNGGGKQALETVQRLLPVLCQDHGLTPDQVVAIASNIGGKQALETVQRLLPVLCQDHGLTPDQVVAIASNGGGKQALETVQRLLPVLCQDHGLTPDQVVAIASNGGGKQALETVQRLLPVLCQDHGLTPDQVVAIASHDGGKQALETVQRLLPVLCQDHGLTPDQVVAIASHDGGKQALETVQRLLPVLCQDHGLTPDQVVAIASNIGGKQALETVQRLLPVLCQDHGLTPDQVVAIASHDGGKQALETVQRLLPVLCQDHGLTPDQVVAIASNKGGKQALETVQRLLPVLCQDHGLTPDQVVAIASNGGGKQALESIVAQLSRPDPALAALTNDHLVALACLGGRPAMDAVKKGLPHAPELIRRVNRRIGERTSHRVAGSTGGGGGSGTASSKGGRADPAFLYKVVSSSSFEFMVSKGEELFTGVVPILVELDGDVNDHKFSVRGEGEGDATNGKLTLKFICTTGKLPVPWPTLVTTFGYGVACFSRYPDHMKQHDFFKSAMPEGYVQERTISFKDDGTYKTRAEVKFEGDTLVNRIELKGIDFKEDGNILGHKLEYNFNSHNVYITADKQKNGIKANFKIRHNVEDGSVQLADHYQQNTPIGDGPVLLPDNHYLSHQSKLSKDPNEKRDHMVLLEFVTAAGITHGMDELYKVDMDSATHIKFSKRDEDGKELAGATMELRDSSGKTISTWISDGQVKDFYLYPGKYTFVETAAPDGYEVATAITFTVNEQGQVTVNGKATKGDAHIGS

SEQ ID NO: 55 - RNA, 3798 nt, synthetic construct
  source 1..3798: mol_type = other RNA
gcgaattaattcgagctcggtacccagcttgcttgttctttttgcagaagctcagaataaacgctcaactttggcagatcaattccccggtgctagcatgggttccgcccacatcgtgatggtggacgcctacaagccgacgaagaccggtacaagtttgtacaaaaaagcaggctccgcggccgcccccttcaccatgcaggtggatctacgcacgctcggctacagtcagcagcagcaagagaagatcaaaccgaaggtgcgttcgacagtggcgcagcaccacgaggcactggtgggccatgggtttacacacgcgcacatcgttgcgctcagccaacacccggcagcgttagggaccgtcgctgtcacgtatcagcacataatcacggcgttgccagaggcgacacacgaagacatcgttggcgtcggcaaacagtggtccggcgcacgcgccctggaggccttgctcacggatgcgggggagttgagaggtccgccgttacagttggacacaggccaacttgtgaagattgcaaaacgtggcggcgtgaccgcaatggaggcagtgcatgcatcgcgcaatgcactgacgggtgcccccctgaacctgaccccggaccaagtggtggctatcgccagcaacggtggcggcaagcaagcgctcgaaacggtgcagcggctgttgccggtgctgtgccaggaccatggcctgaccccggaccaagtggtggctatcgccagcaacaagggcggcaagcaagcgctcgaaacggtgcagcggctgttgccggtgctgtgccaggaccatggcctgactccggaccaagtggtggctatcgccagccacgatggcggcaagcaagcgctcgaaacggtgcagcggctgttgccggtgctgtgccaggaccatggcctgactccggaccaagtggtggctatcgccagccacgatggcggcaagcaagcgctcgaaacggtgcagcggctgttgccggtgctgtgccaggaccatggcctgaccccggaccaagtggtggctatcgccagcaacattggcggcaagcaagcgctcgaaacggtgcagcggctgttgccggtgctgtgccaggaccatggcctgaccccggaccaagtggtggctatcgccagcaacggtggcggcaagcaagcgctcgaaacggtgcagcggctgttgccggtgctgtgccaggaccatggcctgaccccggaccaagtggtggctatcgccagcaacattggcggcaagcaagcgctcgaaacggtgcagcggctgttgccggtgctgtgccaggaccatggcctgaccccggaccaagtggtggctatcgccagcaacggtggcggcaagcaagcgctcgaaacggtgcagcggctgttgccggtgctgtgccaggaccatggcctgaccccggaccaagtggtggctatcgccagcaacggtggcggcaagcaagcgctcgaaacggtgcagcggctgttgccggtgctgtgccaggaccatggcctgactccggaccaagtggtggctatcgccagccacgatggcggcaagcaagcgctcgaaacggtgcagcggctgttgccggtgctgtgccaggaccatggcctgaccccggaccaagtggtggctatcgccagccacgatggcggcaagcaagcgctcgaaacggtgcagcggctgttgccggtgctgtgccaggaccatggcctgaccccggaccaagtggtggctatcgccagcaacattggcggcaagcaagcgctcgaaacggtgcagcggctgttgccggtgctgtgccaggaccatggcctgactccggaccaagtggtggctatcgccagccacgatggcggcaagcaagcgctcgaaacggtgcagcggctgttgccggtgctgtgccaggaccatggcctgaccccggaccaagtggtggctatcgccagcaacaagggcggcaagcaagcgctcgaaacggtgcagcggctgttgccggtgctgtgccaggaccatggcctgaccccggaccaagtggtggctatcgccagcaacggtggcggcaagcaagcgctcgaaagcattgtggcccagctgagccggcctgatccggcgttggccgcgttgaccaacgaccacctcgtcgccttggcctgcctcggcggacgtcctgccatggatgcagtgaaaaagggattgccgcacgcgccggaattgatcagaagagtcaatcgccgtattggcgaacgcacgtcccatcgcgttgcgggatccactggaggcggaggtggctccggcaccgcctcctccaccggtatggtgagcaagggcgaggaggataacatggccatcatcaaggagttcatgcgcttcaaggtgcacatggagggctccgtgaacggccacgagttcgagatcgagggcgagggcgagggccgcccctacgagggcacccagaccgccaagctgaaggtgaccaagggtggccccctgcccttcgcctgggacatcctgtcccctcagttcatgtacggctccaaggcctacgtgaagcaccccgccgacatccccgactacttgaagctgtccttccccgagggcttcaagtgggagcgcgtgatgaacttcgaggacggcggcgtggtgaccgtgacccaggactcctccctgcaggacggcgagttcatctacaaggtgaagctgcgcggcaccaacttcccctccgacggccccgtaatgcagaagaagaccatgggctgggaggcctcctccgagcggatgtaccccgaggacggcgccctgaagggcgagatcaagcagaggctgaagctgaaggacggcggccactacgacgctgaggtcaagaccacctacaaggccaagaagcccgtgcagctgcccggcgcctacaacgtcaacatcaagttggacatcacctcccacaacgaggactacaccatcgtggaacagtacgaacgcgccgagggccgccactccaccggcggcatggacgagctgtacaagggtacaagtttgtacaaaaaagcaggctccgcggccgcccccttcaccatgctcagacaaaggccacagctggagactgaggagacagtggaggaagagagagcagcagatgaggaagagaggagaaagactgaagctctgagcgagatcgaggttctgagggaggcccaggagcccagtggtcccctcatgctgtcttcagagctctccctagaagcagcagaagatgaaaagtctcgtactagcctcatccccccagaatggtgggcctggtctgaggaggggcagcccgagccccctgcactgcccatgctgcctgaacttcctgaagtgcccatggagatgcccccaaggcctgaactctcttcagaggctaagggtgggcgcgccgacccagctttcttgtacaaagtggtaagcttaggttccgcccatatagttatggtggacgcctataaacccactaagagtcgacggcccgggatcctgtacaagtaaagcggccgctctagataaatgatagcttgatctggttaccactaaaccagcctcaagaacacccgaatggagtctctaagctacataataccaacttacactttacaaaatgttgtcccccaaaatgtagccattcgtatctgctcctaataaaaagaaagtttcttcacattctaaaaaaaaaaaaaaaaaaaaaaaaaaaaaaaaaaccccccccccccccccctgcaggcgcgccgccggcgatttaaattaat

SEQ ID NO: 56 - protein, 1147 aa, synthetic construct
MGSAHIVMVDAYKPTKTGTSLYKKAGSAAAPFTMQVDLRTLGYSQQQQEKIKPKVRSTVAQHHEALVGHGFTHAHIVALSQHPAALGTVAVTYQHIITALPEATHEDIVGVGKQWSGARALEALLTDAGELRGPPLQLDTGQLVKIAKRGGVTAMEAVHASRNALTGAPLNLTPDQVVAIASNGGGKQALETVQRLLPVLCQDHGLTPDQVVAIASNKGGKQALETVQRLLPVLCQDHGLTPDQVVAIASHDGGKQALETVQRLLPVLCQDHGLTPDQVVAIASHDGGKQALETVQRLLPVLCQDHGLTPDQVVAIASNIGGKQALETVQRLLPVLCQDHGLTPDQVVAIASNGGGKQALETVQRLLPVLCQDHGLTPDQVVAIASNIGGKQALETVQRLLPVLCQDHGLTPDQVVAIASNGGGKQALETVQRLLPVLCQDHGLTPDQVVAIASNGGGKQALETVQRLLPVLCQDHGLTPDQVVAIASHDGGKQALETVQRLLPVLCQDHGLTPDQVVAIASHDGGKQALETVQRLLPVLCQDHGLTPDQVVAIASNIGGKQALETVQRLLPVLCQDHGLTPDQVVAIASHDGGKQALETVQRLLPVLCQDHGLTPDQVVAIASNKGGKQALETVQRLLPVLCQDHGLTPDQVVAIASNGGGKQALESIVAQLSRPDPALAALTNDHLVALACLGGRPAMDAVKKGLPHAPELIRRVNRRIGERTSHRVAGSTGGGGGSGTASSTGMVSKGEEDNMAIIKEFMRFKVHMEGSVNGHEFEIEGEGEGRPYEGTQTAKLKVTKGGPLPFAWDILSPQFMYGSKAYVKHPADIPDYLKLSFPEGFKWERVMNFEDGGVVTVTQDSSLQDGEFIYKVKLRGTNFPSDGPVMQKKTMGWEASSERMYPEDGALKGEIKQRLKLKDGGHYDAEVKTTYKAKKPVQLPGAYNVNIKLDITSHNEDYTIVEQYERAEGRHSTGGMDELYKGTSLYKKAGSAAAPFTMLRQRPQLETEETVEEERAADEEERRKTEALSEIEVLREAQEPSGPLMLSSELSLEAAEDEKSRTSLIPPEWWAWSEEGQPEPPALPMLPELPEVPMEMPPRPELSSEAKGGRADPAFLYKVVSLGSAHIVMVDAYKPTKSRRPGILYK

SEQ ID NO: 57 - RNA, 4976 nt, synthetic construct
  source 1..4976: mol_type = other RNA
gcgaattaattcgagctcggtacccagcttgcttgttctttttgcagaagctcagaataaacgctcaactttggcagatcaattccccggtgctagcatggatagtgctacccatattaaattctcaaaacgtgatgaggacggcaaagagttagctggtgcaactatggagttgcgtgattcatctggtaaaactattagtacatggatttcagatggacaagtgaaagatttctacctgtatccaggaaaatatacatttgtcgaaaccgcagcaccagacggttatgaggtagcaactgctattacctttacagttaatgagcaaggtcaggttactgtaaatggcaaagcaactaaaggtgacgctcatattggatccaccggtacaagtttgtacaaaaaagcaggctccgcggccgcccccttcaccatgcaggtggatctacgcacgctcggctacagtcagcagcagcaagagaagatcaaaccgaaggtgcgttcgacagtggcgcagcaccacgaggcactggtgggccatgggtttacacacgcgcacatcgttgcgctcagccaacacccggcagcgttagggaccgtcgctgtcacgtatcagcacataatcacggcgttgccagaggcgacacacgaagacatcgttggcgtcggcaaacagtggtccggcgcacgcgccctggaggccttgctcacggatgcgggggagttgagaggtccgccgttacagttggacacaggccaacttgtgaagattgcaaaacgtggcggcgtgaccgcaatggaggcagtgcatgcatcgcgcaatgcactgacgggtgcccccctgaacctgaccccggaccaagtggtggctatcgccagcaacggtggcggcaagcaagcgctcgaaacggtgcagcggctgttgccggtgctgtgccaggaccatggcctgaccccggaccaagtggtggctatcgccagcaacaagggcggcaagcaagcgctcgaaacggtgcagcggctgttgccggtgctgtgccaggaccatggcctgactccggaccaagtggtggctatcgccagccacgatggcggcaagcaagcgctcgaaacggtgcagcggctgttgccggtgctgtgccaggaccatggcctgactccggaccaagtggtggctatcgccagccacgatggcggcaagcaagcgctcgaaacggtgcagcggctgttgccggtgctgtgccaggaccatggcctgaccccggaccaagtggtggctatcgccagcaacattggcggcaagcaagcgctcgaaacggtgcagcggctgttgccggtgctgtgccaggaccatggcctgaccccggaccaagtggtggctatcgccagcaacggtggcggcaagcaagcgctcgaaacggtgcagcggctgttgccggtgctgtgccaggaccatggcctgaccccggaccaagtggtggctatcgccagcaacattggcggcaagcaagcgctcgaaacggtgcagcggctgttgccggtgctgtgccaggaccatggcctgaccccggaccaagtggtggctatcgccagcaacggtggcggcaagcaagcgctcgaaacggtgcagcggctgttgccggtgctgtgccaggaccatggcctgaccccggaccaagtggtggctatcgccagcaacggtggcggcaagcaagcgctcgaaacggtgcagcggctgttgccggtgctgtgccaggaccatggcctgactccggaccaagtggtggctatcgccagccacgatggcggcaagcaagcgctcgaaacggtgcagcggctgttgccggtgctgtgccaggaccatggcctgaccccggaccaagtggtggctatcgccagccacgatggcggcaagcaagcgctcgaaacggtgcagcggctgttgccggtgctgtgccaggaccatggcctgaccccggaccaagtggtggctatcgccagcaacattggcggcaagcaagcgctcgaaacggtgcagcggctgttgccggtgctgtgccaggaccatggcctgactccggaccaagtggtggctatcgccagccacgatggcggcaagcaagcgctcgaaacggtgcagcggctgttgccggtgctgtgccaggaccatggcctgaccccggaccaagtggtggctatcgccagcaacaagggcggcaagcaagcgctcgaaacggtgcagcggctgttgccggtgctgtgccaggaccatggcctgaccccggaccaagtggtggctatcgccagcaacggtggcggcaagcaagcgctcgaaagcattgtggcccagctgagccggcctgatccggcgttggccgcgttgaccaacgaccacctcgtcgccttggcctgcctcggcggacgtcctgccatggatgcagtgaaaaagggattgccgcacgcgccggaattgatcagaagagtcaatcgccgtattggcgaacgcacgtcccatcgcgttgcgggatccactggaggcggaggtggctccggcaccgcctcctccaccggtatggtgagcaagggcgaggaggataacatggccatcatcaaggagttcatgcgcttcaaggtgcacatggagggctccgtgaacggccacgagttcgagatcgagggcgagggcgagggccgcccctacgagggcacccagaccgccaagctgaaggtgaccaagggtggccccctgcccttcgcctgggacatcctgtcccctcagttcatgtacggctccaaggcctacgtgaagcaccccgccgacatccccgactacttgaagctgtccttccccgagggcttcaagtgggagcgcgtgatgaacttcgaggacggcggcgtggtgaccgtgacccaggactcctccctgcaggacggcgagttcatctacaaggtgaagctgcgcggcaccaacttcccctccgacggccccgtaatgcagaagaagaccatgggctgggaggcctcctccgagcggatgtaccccgaggacggcgccctgaagggcgagatcaagcagaggctgaagctgaaggacggcggccactacgacgctgaggtcaagaccacctacaaggccaagaagcccgtgcagctgcccggcgcctacaacgtcaacatcaagttggacatcacctcccacaacgaggactacaccatcgtggaacagtacgaacgcgccgagggccgccactccaccggcggcatggacgagctgtacaagggtacaagtttgtacaaaaaagcaggctccgcggccgcccccttcaccatgctcagacaaaggccacagctggagactgaggagacagtggaggaagagagagcagcagatgaggaagagaggagaaagactgaagctctgagcgagatcgaggttctgagggaggcccaggagcccagtggtcccctcatgctgtcttcagagctctccctagaagcagcagaagatgaaaagtctcgtactagcctcatccccccagaatggtgggcctggtctgaggaggggcagcccgagccccctgcactgcccatgctgcctgaacttcctgaagtgcccatggagatgcccccaaggcctgaactctcttcagaggctaagggtgggcgcgccgacccagctttcttgtacaaagtggtaagcttcgaattcatggtgagcaagggcgaggagctgttcaccggggtggtgcccatcctggtcgagctggacggcgacgtaaacggccacaagttcagcgtccgcggcgagggcgagggcgatgccaccaacggcaagctgaccctgaagttcatctgcaccaccggcaagctgcccgtgccctggcccaccctcgtgaccaccttcggctacggcgtggcctgcttcagccgctaccccgaccacatgaagcagcacgacttcttcaagtccgccatgcccgaaggctacgtccaggagcgcaccatctctttcaaggacgacggtacctacaagacccgcgccgaggtgaagttcgagggcgacaccctggtgaaccgcatcgagctgaagggcatcgacttcaaggaggacggcaacatcctggggcacaagctggagtacaacttcaacagccacaacgtctatatcacggccgacaagcagaagaacggcatcaaggctaacttcaagatccgccacaacgttgaggacggcagcgtgcagctcgccgaccactaccagcagaacacccccatcggcgacggccccgtgctgctgcccgacaaccactacctgagccatcagtccaagctgagcaaagaccccaacgagaagcgcgatcacatggtcctgctggagttcgtgaccgccgccgggattacacatggcatggacgagctgtacaaggtcgacatggatagtgctacccatattaaattctcaaaacgtgatgaggacggcaaagagttagctggtgcaactatggagttgcgtgattcatctggtaaaactattagtacatggatttcagatggacaagtgaaagatttctacctgtatccaggaaaatatacatttgtcgaaaccgcagcaccagacggttatgaggtagcaactgctattacctttacagttaatgagcaaggtcaggttactgtaaatggcaaagcaactaaaggtgacgctcatattggatcctaagcggccgctctagataaatgatagcttgatctggttaccactaaaccagcctcaagaacacccgaatggagtctctaagctacataataccaacttacactttacaaaatgttgtcccccaaaatgtagccattcgtatctgctcctaataaaaagaaagtttcttcacattctaaaaaaaaaaaaaaaaaaaaaaaaaaaaaaaaaaccccccccccccccccctgcaggcgcgccgccggcgatttaaattaat

SEQ ID NO: 58 - protein, 1540 aa, synthetic construct
MDSATHIKFSKRDEDGKELAGATMELRDSSGKTISTWISDGQVKDFYLYPGKYTFVETAAPDGYEVATAITFTVNEQGQVTVNGKATKGDAHIGSTGTSLYKKAGSAAAPFTMQVDLRTLGYSQQQQEKIKPKVRSTVAQHHEALVGHGFTHAHIVALSQHPAALGTVAVTYQHIITALPEATHEDIVGVGKQWSGARALEALLTDAGELRGPPLQLDTGQLVKIAKRGGVTAMEAVHASRNALTGAPLNLTPDQVVAIASNGGGKQALETVQRLLPVLCQDHGLTPDQVVAIASNKGGKQALETVQRLLPVLCQDHGLTPDQVVAIASHDGGKQALETVQRLLPVLCQDHGLTPDQVVAIASHDGGKQALETVQRLLPVLCQDHGLTPDQVVAIASNIGGKQALETVQRLLPVLCQDHGLTPDQVVAIASNGGGKQALETVQRLLPVLCQDHGLTPDQVVAIASNIGGKQALETVQRLLPVLCQDHGLTPDQVVAIASNGGGKQALETVQRLLPVLCQDHGLTPDQVVAIASNGGGKQALETVQRLLPVLCQDHGLTPDQVVAIASHDGGKQALETVQRLLPVLCQDHGLTPDQVVAIASHDGGKQALETVQRLLPVLCQDHGLTPDQVVAIASNIGGKQALETVQRLLPVLCQDHGLTPDQVVAIASHDGGKQALETVQRLLPVLCQDHGLTPDQVVAIASNKGGKQALETVQRLLPVLCQDHGLTPDQVVAIASNGGGKQALESIVAQLSRPDPALAALTNDHLVALACLGGRPAMDAVKKGLPHAPELIRRVNRRIGERTSHRVAGSTGGGGGSGTASSTGMVSKGEEDNMAIIKEFMRFKVHMEGSVNGHEFEIEGEGEGRPYEGTQTAKLKVTKGGPLPFAWDILSPQFMYGSKAYVKHPADIPDYLKLSFPEGFKWERVMNFEDGGVVTVTQDSSLQDGEFIYKVKLRGTNFPSDGPVMQKKTMGWEASSERMYPEDGALKGEIKQRLKLKDGGHYDAEVKTTYKAKKPVQLPGAYNVNIKLDITSHNEDYTIVEQYERAEGRHSTGGMDELYKGTSLYKKAGSAAAPFTMLRQRPQLETEETVEEERAADEEERRKTEALSEIEVLREAQEPSGPLMLSSELSLEAAEDEKSRTSLIPPEWWAWSEEGQPEPPALPMLPELPEVPMEMPPRPELSSEAKGGRADPAFLYKVVSFEFMVSKGEELFTGVVPILVELDGDVNGHKFSVRGEGEGDATNGKLTLKFICTTGKLPVPWPTLVTTFGYGVACFSRYPDHMKQHDFFKSAMPEGYVQERTISFKDDGTYKTRAEVKFEGDTLVNRIELKGIDFKEDGNILGHKLEYNFNSHNVYITADKQKNGIKANFKIRHNVEDGSVQLADHYQQNTPIGDGPVLLPDNHYLSHQSKLSKDPNEKRDHMVLLEFVTAAGITHGMDELYKVDMDSATHIKFSKRDEDGKELAGATMELRDSSGKTISTWISDGQVKDFYLYPGKYTFVETAAPDGYEVATAITFTVNEQGQVTVNGKATKGDAHIGS

SEQ ID NO: 59 - DNA, 3435 bp, synthetic construct
  source 1..3435: mol_type = other DNA
atgggttccgcccacatcgtgatggtggacgcctacaagccgacgaagaccggtacaagtttgtacaaaaaagcaggctccgcggccgcccccttcaccatggtagatttgagaactttgggatattcacagcagcagcaggaaaagatcaagcccaaagtgaggtcgacagtcgcgcagcatcacgaagcgctggtgggtcatgggtttacacatgcccacatcgtagccttgtcgcagcaccctgcagcccttggcacggtcgccgtcaagtaccaggacatgattgcggcgttgccggaagccacacatgaggcgatcgtcggtgtggggaaacagtggagcggagcccgagcgcttgaggccctgttgacggtcgcgggagagctgagagggcctccccttcagctggacacgggccagttgctgaagatcgcgaagcggggaggagtcacggcggtcgaggcggtgcacgcgtggcgcaatgcgctcacgggagcacccctcaacctgaccccagagcaggtcgtggcaattgcgagccatgacgggggaaagcaggcactcgaaaccgtccagaggttgctgcctgtgctgtgccaagcgcacggacttacgccagagcaggtcgtggcaattgcgagccatgacgggggaaagcaggcactcgaaaccgtccagaggttgctgcctgtgctgtgccaagcgcacggactaaccccagagcaggtcgtggcaattgcgagcaacatcgggggaaagcaggcactcgaaaccgtccagaggttgctgcctgtgctgtgccaagcgcacgggttgaccccagagcaggtcgtggcaattgcgagcaacggagggggaaagcaggcactcgaaaccgtccagaggttgctgcctgtgctgtgccaagcgcacgggttgaccccagagcaggtcgtggcaattgcgagcaacggagggggaaagcaggcactcgaaaccgtccagaggttgctgcctgtgctgtgccaagcgcacggactgacaccagagcaggtcgtggcaattgcgagccatgacgggggaaagcaggcactcgaaaccgtccagaggttgctgcctgtgctgtgccaagcgcacggacttacacccgaacaagtcgtggcaattgcgagccatgacgggggaaagcaggcactcgaaaccgtccagaggttgctgcctgtgctgtgccaagcgcacggactaaccccagagcaggtcgtggcaattgcgagcaacatcgggggaaagcaggcactcgaaaccgtccagaggttgctgcctgtgctgtgccaagcgcacgggttgaccccagagcaggtcgtggcaattgcgagcaacggagggggaaagcaggcactcgaaaccgtccagaggttgctgcctgtgctgtgccaagcgcacgggttgaccccagagcaggtcgtggcaattgcgagcaacggagggggaaagcaggcactcgaaaccgtccagaggttgctgcctgtgctgtgccaagcgcacggactgacaccagagcaggtcgtggcaattgcgagccatgacgggggaaagcaggcactcgaaaccgtccagaggttgctgcctgtgctgtgccaagcgcacggacttacacccgaacaagtcgtggcaattgcgagccatgacgggggaaagcaggcactcgaaaccgtccagaggttgctgcctgtgctgtgccaagcgcacggcctcaccccagagcaggtcgtggcaattgcgagcaacatcgggggaaagcaggcactcgaaaccgtccagaggttgctgcctgtgctgtgccaagcgcacggacttacgccagagcaggtcgtggcaattgcgagcaacggagggggaaagcaggcactcgaaaccgtccagaggttgctgcctgtgctgtgccaagcgcacggactaaccccagagcaggtcgtggcaattgcgagcaacggagggggaaagcaggcactcgaaaccgtccagaggttgctgcctgtgctgtgccaagcgcacgggttgaccccagagcaggtcgtggcaattgcgagccatgacgggggaaagcaggcactcgaaaccgtccagaggttgctgcctgtgctgtgccaagcgcacggcctgaccccagagcaggtcgtggcaattgcgagccatgacgggggaaagcaggcactcgaaaccgtccagaggttgctgcctgtgctgtgccaagcgcacggactgacaccagagcaggtcgtggcaattgcgagcaacatcgggggaaagcaggcactcgaaaccgtccagaggttgctgcctgtgctgtgccaagcgcacggactcacgcctgagcaggtagtggctattgcatccaacggagggggcagacccgcactggagtcaatcgtggcccagctttcgaggccggaccccgcgctggccgcactcactaatgatcatcttgtagcgctggcctgcctcggcggacgacccgccttggatgcggtgaagaaggggctcccgcacgcgcctgcattgattaagcggaccaacagaaggattcccgagaggacatcacatcgagtggcaaagggtgggcgcgccgacccagctttcttgtacaaagtggtctcgagaatggtgagcaagggcgaggaggataacatggccatcatcaaggagttcatgcgcttcaaggtgcacatggagggctccgtgaacggccacgagttcgagatcgagggcgagggcgagggccgcccctacgagggcacccagaccgccaagctgaaggtgaccaagggtggccccctgcccttcgcctgggacatcctgtcccctcagttcatgtacggctccaaggcctacgtgaagcaccccgccgacatccccgactacttgaagctgtccttccccgagggcttcaagtgggagcgcgtgatgaacttcgaggacggcggcgtggtgaccgtgacccaggactcctccctgcaggacggcgagttcatctacaaggtgaagctgcgcggcaccaacttcccctccgacggccccgtaatgcagaagaagaccatgggctgggaggcctcctccgagcggatgtaccccgaggacggcgccctgaagggcgagatcaagcagaggctgaagctgaaggacggcggccactacgacgctgaggtcaagaccacctacaaggccaagaagcccgtgcagctgcccggcgcctacaacgtcaacatcaagttggacatcacctcccacaacgaggactacaccatcgtggaacagtacgaacgcgccgagggccgccactccaccggcggcatggacgagctgtacaagaaaagcttaggttccgcccatatagttatggtggacgcctataaacccactaagagtcgacggcccgggatcctgtacaagtaa

SEQ ID NO: 60 - protein, 1144 aa, synthetic construct
MGSAHIVMVDAYKPTKTGTSLYKKAGSAAAPFTMVDLRTLGYSQQQQEKIKPKVRSTVAQHHEALVGHGFTHAHIVALSQHPAALGTVAVKYQDMIAALPEATHEAIVGVGKQWSGARALEALLTVAGELRGPPLQLDTGQLLKIAKRGGVTAVEAVHAWRNALTGAPLNLTPEQVVAIASHDGGKQALETVQRLLPVLCQAHGLTPEQVVAIASHDGGKQALETVQRLLPVLCQAHGLTPEQVVAIASNIGGKQALETVQRLLPVLCQAHGLTPEQVVAIASNGGGKQALETVQRLLPVLCQAHGLTPEQVVAIASNGGGKQALETVQRLLPVLCQAHGLTPEQVVAIASHDGGKQALETVQRLLPVLCQAHGLTPEQVVAIASHDGGKQALETVQRLLPVLCQAHGLTPEQVVAIASNIGGKQALETVQRLLPVLCQAHGLTPEQVVAIASNGGGKQALETVQRLLPVLCQAHGLTPEQVVAIASNGGGKQALETVQRLLPVLCQAHGLTPEQVVAIASHDGGKQALETVQRLLPVLCQAHGLTPEQVVAIASHDGGKQALETVQRLLPVLCQAHGLTPEQVVAIASNIGGKQALETVQRLLPVLCQAHGLTPEQVVAIASNGGGKQALETVQRLLPVLCQAHGLTPEQVVAIASNGGGKQALETVQRLLPVLCQAHGLTPEQVVAIASHDGGKQALETVQRLLPVLCQAHGLTPEQVVAIASHDGGKQALETVQRLLPVLCQAHGLTPEQVVAIASNIGGKQALETVQRLLPVLCQAHGLTPEQVVAIASNGGGRPALESIVAQLSRPDPALAALTNDHLVALACLGGRPALDAVKKGLPHAPALIKRTNRRIPERTSHRVAKGGRADPAFLYKVVSRMVSKGEEDNMAIIKEFMRFKVHMEGSVNGHEFEIEGEGEGRPYEGTQTAKLKVTKGGPLPFAWDILSPQFMYGSKAYVKHPADIPDYLKLSFPEGFKWERVMNFEDGGVVTVTQDSSLQDGEFIYKVKLRGTNFPSDGPVMQKKTMGWEASSERMYPEDGALKGEIKQRLKLKDGGHYDAEVKTTYKAKKPVQLPGAYNVNIKLDITSHNEDYTIVEQYERAEGRHSTGGMDELYKKSLGSAHIVMVDAYKPTKSRRPGILYK

SEQ ID NO: 61 - DNA, 3948 bp, synthetic construct
  source 1..3948: mol_type = other DNA
atgacaactgaagaagatagtgctacccatattaaattctcaaaacgtgatgaggacggccgtgagttagctggtgcaactatggagttgcgtgattcatctggtaaaactattagtacatggatttcagatggacatgtgaaggatttctacctgtatccaggaaaatatacatttgtcgaaaccgcagcaccagacggttatgaggtagcaactccaattgaatttacagttaatgaggacggtcaggttactgtagatggtgaagcaactgaaggtgacgctcatactggatccagtggtagcaccggtacaagtttgtacaaaaaagcaggctccgcggccgcccccttcaccatggtagatttgagaactttgggatattcacagcagcagcaggaaaagatcaagcccaaagtgaggtcgacagtcgcgcagcatcacgaagcgctggtgggtcatgggtttacacatgcccacatcgtagccttgtcgcagcaccctgcagcccttggcacggtcgccgtcaagtaccaggacatgattgcggcgttgccggaagccacacatgaggcgatcgtcggtgtggggaaacagtggagcggagcccgagcgcttgaggccctgttgacggtcgcgggagagctgagagggcctccccttcagctggacacgggccagttgctgaagatcgcgaagcggggaggagtcacggcggtcgaggcggtgcacgcgtggcgcaatgcgctcacgggagcacccctcaacctgaccccagagcaggtcgtggcaattgcgagccatgacgggggaaagcaggcactcgaaaccgtccagaggttgctgcctgtgctgtgccaagcgcacggacttacgccagagcaggtcgtggcaattgcgagccatgacgggggaaagcaggcactcgaaaccgtccagaggttgctgcctgtgctgtgccaagcgcacggactaaccccagagcaggtcgtggcaattgcgagcaacatcgggggaaagcaggcactcgaaaccgtccagaggttgctgcctgtgctgtgccaagcgcacgggttgaccccagagcaggtcgtggcaattgcgagcaacggagggggaaagcaggcactcgaaaccgtccagaggttgctgcctgtgctgtgccaagcgcacgggttgaccccagagcaggtcgtggcaattgcgagcaacggagggggaaagcaggcactcgaaaccgtccagaggttgctgcctgtgctgtgccaagcgcacggactgacaccagagcaggtcgtggcaattgcgagccatgacgggggaaagcaggcactcgaaaccgtccagaggttgctgcctgtgctgtgccaagcgcacggacttacacccgaacaagtcgtggcaattgcgagccatgacgggggaaagcaggcactcgaaaccgtccagaggttgctgcctgtgctgtgccaagcgcacggactaaccccagagcaggtcgtggcaattgcgagcaacatcgggggaaagcaggcactcgaaaccgtccagaggttgctgcctgtgctgtgccaagcgcacgggttgaccccagagcaggtcgtggcaattgcgagcaacggagggggaaagcaggcactcgaaaccgtccagaggttgctgcctgtgctgtgccaagcgcacgggttgaccccagagcaggtcgtggcaattgcgagcaacggagggggaaagcaggcactcgaaaccgtccagaggttgctgcctgtgctgtgccaagcgcacggactgacaccagagcaggtcgtggcaattgcgagccatgacgggggaaagcaggcactcgaaaccgtccagaggttgctgcctgtgctgtgccaagcgcacggacttacacccgaacaagtcgtggcaattgcgagccatgacgggggaaagcaggcactcgaaaccgtccagaggttgctgcctgtgctgtgccaagcgcacggcctcaccccagagcaggtcgtggcaattgcgagcaacatcgggggaaagcaggcactcgaaaccgtccagaggttgctgcctgtgctgtgccaagcgcacggacttacgccagagcaggtcgtggcaattgcgagcaacggagggggaaagcaggcactcgaaaccgtccagaggttgctgcctgtgctgtgccaagcgcacggactaaccccagagcaggtcgtggcaattgcgagcaacggagggggaaagcaggcactcgaaaccgtccagaggttgctgcctgtgctgtgccaagcgcacgggttgaccccagagcaggtcgtggcaattgcgagccatgacgggggaaagcaggcactcgaaaccgtccagaggttgctgcctgtgctgtgccaagcgcacggcctgaccccagagcaggtcgtggcaattgcgagccatgacgggggaaagcaggcactcgaaaccgtccagaggttgctgcctgtgctgtgccaagcgcacggactgacaccagagcaggtcgtggcaattgcgagcaacatcgggggaaagcaggcactcgaaaccgtccagaggttgctgcctgtgctgtgccaagcgcacggactcacgcctgagcaggtagtggctattgcatccaacggagggggcagacccgcactggagtcaatcgtggcccagctttcgaggccggaccccgcgctggccgcactcactaatgatcatcttgtagcgctggcctgcctcggcggacgacccgccttggatgcggtgaagaaggggctcccgcacgcgcctgcattgattaagcggaccaacagaaggattcccgagaggacatcacatcgagtggcaaagggtgggcgcgccgacccagctttcttgtacaaagtggtctcgagctcaagcttcgaattcatggtgagcaagggcgaggagctgttcaccggggtggtgcccatcctggtcgagctggacggcgacgtaaacgaccacaagttcagcgtccgcggcgagggcgagggcgatgccaccaacggcaagctgaccctgaagttcatctgcaccaccggcaagctgcccgtgccctggcccaccctcgtgaccaccttcggctacggcgtggcctgcttcagccgctaccccgaccacatgaagcagcacgacttcttcaagtccgccatgcccgaaggctacgtccaggagcgcaccatctctttcaaggacgacggtacctacaagacccgcgccgaggtgaagttcgagggcgacaccctggtgaaccgcatcgagctgaagggcatcgacttcaaggaggacggcaacatcctggggcacaagctggagtacaacttcaacagccacaacgtctatatcacggccgacaagcagaagaacggcatcaaggctaacttcaagatccgccacaacgttgaggacggcagcgtgcagctcgccgaccactaccagcagaacacccccatcggcgacggccccgtgctgctgcccgacaaccactacctgagccatcagtccaagctgagcaaagaccccaacgagaagcgcgatcacatggtcctgctggagttcgtgaccgccgccgggattacacatggcatggacgagctgtacaaggtcgacatgacaactgaagaagatagtgctacccatattaaattctcaaaacgtgatgaggacggccgtgagttagctggtgcaactatggagttgcgtgattcatctggtaaaactattagtacatggatttcagatggacatgtgaaggatttctacctgtatccaggaaaatatacatttgtcgaaaccgcagcaccagacggttatgaggtagcaactccaattgaatttacagttaatgaggacggtcaggttactgtagatggtgaagcaactgaaggtgacgctcatactggatccagtggtagctaa

SEQ ID NO: 62 - protein, 1315 aa, synthetic construct
MTTEEDSATHIKFSKRDEDGRELAGATMELRDSSGKTISTWISDGHVKDFYLYPGKYTFVETAAPDGYEVATPIEFTVNEDGQVTVDGEATEGDAHTGSSGSTGTSLYKKAGSAAAPFTMVDLRTLGYSQQQQEKIKPKVRSTVAQHHEALVGHGFTHAHIVALSQHPAALGTVAVKYQDMIAALPEATHEAIVGVGKQWSGARALEALLTVAGELRGPPLQLDTGQLLKIAKRGGVTAVEAVHAWRNALTGAPLNLTPEQVVAIASHDGGKQALETVQRLLPVLCQAHGLTPEQVVAIASHDGGKQALETVQRLLPVLCQAHGLTPEQVVAIASNIGGKQALETVQRLLPVLCQAHGLTPEQVVAIASNGGGKQALETVQRLLPVLCQAHGLTPEQVVAIASNGGGKQALETVQRLLPVLCQAHGLTPEQVVAIASHDGGKQALETVQRLLPVLCQAHGLTPEQVVAIASHDGGKQALETVQRLLPVLCQAHGLTPEQVVAIASNIGGKQALETVQRLLPVLCQAHGLTPEQVVAIASNGGGKQALETVQRLLPVLCQAHGLTPEQVVAIASNGGGKQALETVQRLLPVLCQAHGLTPEQVVAIASHDGGKQALETVQRLLPVLCQAHGLTPEQVVAIASHDGGKQALETVQRLLPVLCQAHGLTPEQVVAIASNIGGKQALETVQRLLPVLCQAHGLTPEQVVAIASNGGGKQALETVQRLLPVLCQAHGLTPEQVVAIASNGGGKQALETVQRLLPVLCQAHGLTPEQVVAIASHDGGKQALETVQRLLPVLCQAHGLTPEQVVAIASHDGGKQALETVQRLLPVLCQAHGLTPEQVVAIASNIGGKQALETVQRLLPVLCQAHGLTPEQVVAIASNGGGRPALESIVAQLSRPDPALAALTNDHLVALACLGGRPALDAVKKGLPHAPALIKRTNRRIPERTSHRVAKGGRADPAFLYKVVSSSSFEFMVSKGEELFTGVVPILVELDGDVNDHKFSVRGEGEGDATNGKLTLKFICTTGKLPVPWPTLVTTFGYGVACFSRYPDHMKQHDFFKSAMPEGYVQERTISFKDDGTYKTRAEVKFEGDTLVNRIELKGIDFKEDGNILGHKLEYNFNSHNVYITADKQKNGIKANFKIRHNVEDGSVQLADHYQQNTPIGDGPVLLPDNHYLSHQSKLSKDPNEKRDHMVLLEFVTAAGITHGMDELYKVDMTTEEDSATHIKFSKRDEDGRELAGATMELRDSSGKTISTWISDGHVKDFYLYPGKYTFVETAAPDGYEVATPIEFTVNEDGQVTVDGEATEGDAHTGSSGS

SEQ ID NO: 63 - RNA, 3789 nt, synthetic construct
  source 1..3789: mol_type = other RNA
gcgaattaattcgagctcggtacccagcttgcttgttctttttgcagaagctcagaataaacgctcaactttggcagatcaattccccggtgctagcatgggttccgcccacatcgtgatggtggacgcctacaagccgacgaagaccggtacaagtttgtacaaaaaagcaggctccgcggccgcccccttcaccatggtagatttgagaactttgggatattcacagcagcagcaggaaaagatcaagcccaaagtgaggtcgacagtcgcgcagcatcacgaagcgctggtgggtcatgggtttacacatgcccacatcgtagccttgtcgcagcaccctgcagcccttggcacggtcgccgtcaagtaccaggacatgattgcggcgttgccggaagccacacatgaggcgatcgtcggtgtggggaaacagtggagcggagcccgagcgcttgaggccctgttgacggtcgcgggagagctgagagggcctccccttcagctggacacgggccagttgctgaagatcgcgaagcggggaggagtcacggcggtcgaggcggtgcacgcgtggcgcaatgcgctcacgggagcacccctcaacctgaccccagagcaggtcgtggcaattgcgagccatgacgggggaaagcaggcactcgaaaccgtccagaggttgctgcctgtgctgtgccaagcgcacggacttacgccagagcaggtcgtggcaattgcgagccatgacgggggaaagcaggcactcgaaaccgtccagaggttgctgcctgtgctgtgccaagcgcacggactaaccccagagcaggtcgtggcaattgcgagcaacatcgggggaaagcaggcactcgaaaccgtccagaggttgctgcctgtgctgtgccaagcgcacgggttgaccccagagcaggtcgtggcaattgcgagcaacggagggggaaagcaggcactcgaaaccgtccagaggttgctgcctgtgctgtgccaagcgcacgggttgaccccagagcaggtcgtggcaattgcgagcaacggagggggaaagcaggcactcgaaaccgtccagaggttgctgcctgtgctgtgccaagcgcacggactgacaccagagcaggtcgtggcaattgcgagccatgacgggggaaagcaggcactcgaaaccgtccagaggttgctgcctgtgctgtgccaagcgcacggacttacacccgaacaagtcgtggcaattgcgagccatgacgggggaaagcaggcactcgaaaccgtccagaggttgctgcctgtgctgtgccaagcgcacggactaaccccagagcaggtcgtggcaattgcgagcaacatcgggggaaagcaggcactcgaaaccgtccagaggttgctgcctgtgctgtgccaagcgcacgggttgaccccagagcaggtcgtggcaattgcgagcaacggagggggaaagcaggcactcgaaaccgtccagaggttgctgcctgtgctgtgccaagcgcacgggttgaccccagagcaggtcgtggcaattgcgagcaacggagggggaaagcaggcactcgaaaccgtccagaggttgctgcctgtgctgtgccaagcgcacggactgacaccagagcaggtcgtggcaattgcgagccatgacgggggaaagcaggcactcgaaaccgtccagaggttgctgcctgtgctgtgccaagcgcacggacttacacccgaacaagtcgtggcaattgcgagccatgacgggggaaagcaggcactcgaaaccgtccagaggttgctgcctgtgctgtgccaagcgcacggcctcaccccagagcaggtcgtggcaattgcgagcaacatcgggggaaagcaggcactcgaaaccgtccagaggttgctgcctgtgctgtgccaagcgcacggacttacgccagagcaggtcgtggcaattgcgagcaacggagggggaaagcaggcactcgaaaccgtccagaggttgctgcctgtgctgtgccaagcgcacggactaaccccagagcaggtcgtggcaattgcgagcaacggagggggaaagcaggcactcgaaaccgtccagaggttgctgcctgtgctgtgccaagcgcacgggttgaccccagagcaggtcgtggcaattgcgagccatgacgggggaaagcaggcactcgaaaccgtccagaggttgctgcctgtgctgtgccaagcgcacggcctgaccccagagcaggtcgtggcaattgcgagccatgacgggggaaagcaggcactcgaaaccgtccagaggttgctgcctgtgctgtgccaagcgcacggactgacaccagagcaggtcgtggcaattgcgagcaacatcgggggaaagcaggcactcgaaaccgtccagaggttgctgcctgtgctgtgccaagcgcacggactcacgcctgagcaggtagtggctattgcatccaacggagggggcagacccgcactggagtcaatcgtggcccagctttcgaggccggaccccgcgctggccgcactcactaatgatcatcttgtagcgctggcctgcctcggcggacgacccgccttggatgcggtgaagaaggggctcccgcacgcgcctgcattgattaagcggaccaacagaaggattcccgagaggacatcacatcgagtggcaaagggtgggcgcgccgacccagctttcttgtacaaagtggtctcgagaatggtgagcaagggcgaggaggataacatggccatcatcaaggagttcatgcgcttcaaggtgcacatggagggctccgtgaacggccacgagttcgagatcgagggcgagggcgagggccgcccctacgagggcacccagaccgccaagctgaaggtgaccaagggtggccccctgcccttcgcctgggacatcctgtcccctcagttcatgtacggctccaaggcctacgtgaagcaccccgccgacatccccgactacttgaagctgtccttccccgagggcttcaagtgggagcgcgtgatgaacttcgaggacggcggcgtggtgaccgtgacccaggactcctccctgcaggacggcgagttcatctacaaggtgaagctgcgcggcaccaacttcccctccgacggccccgtaatgcagaagaagaccatgggctgggaggcctcctccgagcggatgtaccccgaggacggcgccctgaagggcgagatcaagcagaggctgaagctgaaggacggcggccactacgacgctgaggtcaagaccacctacaaggccaagaagcccgtgcagctgcccggcgcctacaacgtcaacatcaagttggacatcacctcccacaacgaggactacaccatcgtggaacagtacgaacgcgccgagggccgccactccaccggcggcatggacgagctgtacaagaaaagcttaggttccgcccatatagttatggtggacgcctataaacccactaagagtcgacggcccgggatcctgtacaagtaaagcggccgctctagataaatgatagcttgatctggttaccactaaaccagcctcaagaacacccgaatggagtctctaagctacataataccaacttacactttacaaaatgttgtcccccaaaatgtagccattcgtatctgctcctaataaaaagaaagtttcttcacattctaaaaaaaaaaaaaaaaaaaaaaaaaaaaaaaaaaccccccccccccccccctgcaggcgcgccgccggcgatttaaattaat

SEQ ID NO: 64 - protein, 1144 aa, synthetic construct; identical to SEQ ID NO: 60

SEQ ID NO: 65 - RNA, 4259 nt, synthetic construct
  source 1..4259: mol_type = other RNA
gcgaattaattcgagctcggtacccagcttgcttgttctttttgcagaagctcagaataaacgctcaactttggcagatcaattccccggtgctagcatggatagtgctacccatattaaattctcaaaacgtgatgaggacggcaaagagttagctggtgcaactatggagttgcgtgattcatctggtaaaactattagtacatggatttcagatggacaagtgaaagatttctacctgtatccaggaaaatatacatttgtcgaaaccgcagcaccagacggttatgaggtagcaactgctattacctttacagttaatgagcaaggtcaggttactgtaaatggcaaagcaactaaaggtgacgctcatattggatccaccggtacaagtttgtacaaaaaagcaggctccgcggccgcccccttcaccatggtagatttgagaactttgggatattcacagcagcagcaggaaaagatcaagcccaaagtgaggtcgacagtcgcgcagcatcacgaagcgctggtgggtcatgggtttacacatgcccacatcgtagccttgtcgcagcaccctgcagcccttggcacggtcgccgtcaagtaccaggacatgattgcggcgttgccggaagccacacatgaggcgatcgtcggtgtggggaaacagtggagcggagcccgagcgcttgaggccctgttgacggtcgcgggagagctgagagggcctccccttcagctggacacgggccagttgctgaagatcgcgaagcggggaggagtcacggcggtcgaggcggtgcacgcgtggcgcaatgcgctcacgggagcacccctcaacctgaccccagagcaggtcgtggcaattgcgagccatgacgggggaaagcaggcactcgaaaccgtccagaggttgctgcctgtgctgtgccaagcgcacggacttacgccagagcaggtcgtggcaattgcgagccatgacgggggaaagcaggcactcgaaaccgtccagaggttgctgcctgtgctgtgccaagcgcacggactaaccccagagcaggtcgtggcaattgcgagcaacatcgggggaaagcaggcactcgaaaccgtccagaggttgctgcctgtgctgtgccaagcgcacgggttgaccccagagcaggtcgtggcaattgcgagcaacggagggggaaagcaggcactcgaaaccgtccagaggttgctgcctgtgctgtgccaagcgcacgggttgaccccagagcaggtcgtggcaattgcgagcaacggagggggaaagcaggcactcgaaaccgtccagaggttgctgcctgtgctgtgccaagcgcacggactgacaccagagcaggtcgtggcaattgcgagccatgacgggggaaagcaggcactcgaaaccgtccagaggttgctgcctgtgctgtgccaagcgcacggacttacacccgaacaagtcgtggcaattgcgagccatgacgggggaaagcaggcactcgaaaccgtccagaggttgctgcctgtgctgtgccaagcgcacggactaaccccagagcaggtcgtggcaattgcgagcaacatcgggggaaagcaggcactcgaaaccgtccagaggttgctgcctgtgctgtgccaagcgcacgggttgaccccagagcaggtcgtggcaattgcgagcaacggagggggaaagcaggcactcgaaaccgtccagaggttgctgcctgtgctgtgccaagcgcacgggttgaccccagagcaggtcgtggcaattgcgagcaacggagggggaaagcaggcactcgaaaccgtccagaggttgctgcctgtgctgtgccaagcgcacggactgacaccagagcaggtcgtggcaattgcgagccatgacgggggaaagcaggcactcgaaaccgtccagaggttgctgcctgtgctgtgccaagcgcacggacttacacccgaacaagtcgtggcaattgcgagccatgacgggggaaagcaggcactcgaaaccgtccagaggttgctgcctgtgctgtgccaagcgcacggcctcaccccagagcaggtcgtggcaattgcgagcaacatcgggggaaagcaggcactcgaaaccgtccagaggttgctgcctgtgctgtgccaagcgcacggacttacgccagagcaggtcgtggcaattgcgagcaacggagggggaaagcaggcactcgaaaccgtccagaggttgctgcctgtgctgtgccaagcgcacggactaaccccagagcaggtcgtggcaattgcgagcaacggagggggaaagcaggcactcgaaaccgtccagaggttgctgcctgtgctgtgccaagcgcacgggttgaccccagagcaggtcgtggcaattgcgagccatgacgggggaaagcaggcactcgaaaccgtccagaggttgctgcctgtgctgtgccaagcgcacggcctgaccccagagcaggtcgtggcaattgcgagccatgacgggggaaagcaggcactcgaaaccgtccagaggttgctgcctgtgctgtgccaagcgcacggactgacaccagagcaggtcgtggcaattgcgagcaacatcgggggaaagcaggcactcgaaaccgtccagaggttgctgcctgtgctgtgccaagcgcacggactcacgcctgagcaggtagtggctattgcatccaacggagggggcagacccgcactggagtcaatcgtggcccagctttcgaggccggaccccgcgctggccgcactcactaatgatcatcttgtagcgctggcctgcctcggcggacgacccgccttggatgcggtgaagaaggggctcccgcacgcgcctgcattgattaagcggaccaacagaaggattcccgagaggacatcacatcgagtggcaaagggtgggcgcgccgacccagctttcttgtacaaagtggtctcgagctcaagcttcgaattcatggtgagcaagggcgaggagctgttcaccggggtggtgcccatcctggtcgagctggacggcgacgtaaacgaccacaagttcagcgtccgcggcgagggcgagggcgatgccaccaacggcaagctgaccctgaagttcatctgcaccaccggcaagctgcccgtgccctggcccaccctcgtgaccaccttcggctacggcgtggcctgcttcagccgctaccccgaccacatgaagcagcacgacttcttcaagtccgccatgcccgaaggctacgtccaggagcgcaccatctctttcaaggacgacggtacctacaagacccgcgccgaggtgaagttcgagggcgacaccctggtgaaccgcatcgagctgaagggcatcgacttcaaggaggacggcaacatcctggggcacaagctggagtacaacttcaacagccacaacgtctatatcacggccgacaagcagaagaacggcatcaaggctaacttcaagatccgccacaacgttgaggacggcagcgtgcagctcgccgaccactaccagcagaacacccccatcggcgacggccccgtgctgctgcccgacaaccactacctgagccatcagtccaagctgagcaaagaccccaacgagaagcgcgatcacatggtcctgctggagttcgtgaccgccgccgggattacacatggcatggacgagctgtacaaggtcgacatggatagtgctacccatattaaattctcaaaacgtgatgaggacggcaaagagttagctggtgcaactatggagttgcgtgattcatctggtaaaactattagtacatggatttcagatggacaagtgaaagatttctacctgtatccaggaaaatatacatttgtcgaaaccgcagcaccagacggttatgaggtagcaactgctattacctttacagttaatgagcaaggtcaggttactgtaaatggcaaagcaactaaaggtgacgctcatattggatcctaagcggccgctctagataaatgatagcttgatctggttaccactaaaccagcctcaagaacacccgaatggagtctctaagctacataataccaacttacactttacaaaatgttgtcccccaaaatgtagccattcgtatctgctcctaataaaaagaaagtttcttcacattctaaaaaaaaaaaaaaaaaaaaaaaaaaaaaaaaaaccccccccccccccccctgcaggcgcgccgccggcgatttaaattaat

SEQ ID NO: 66 - protein, 1301 aa, synthetic construct
MDSATHIKFSKRDEDGKELAGATMELRDSSGKTISTWISDGQVKDFYLYPGKYTFVETAAPDGYEVATAITFTVNEQGQVTVNGKATKGDAHIGSTGTSLYKKAGSAAAPFTMVDLRTLGYSQQQQEKIKPKVRSTVAQHHEALVGHGFTHAHIVALSQHPAALGTVAVKYQDMIAALPEATHEAIVGVGKQWSGARALEALLTVAGELRGPPLQLDTGQLLKIAKRGGVTAVEAVHAWRNALTGAPLNLTPEQVVAIASHDGGKQALETVQRLLPVLCQAHGLTPEQVVAIASHDGGKQALETVQRLLPVLCQAHGLTPEQVVAIASNIGGKQALETVQRLLPVLCQAHGLTPEQVVAIASNGGGKQALETVQRLLPVLCQAHGLTPEQVVAIASNGGGKQALETVQRLLPVLCQAHGLTPEQVVAIASHDGGKQALETVQRLLPVLCQAHGLTPEQVVAIASHDGGKQALETVQRLLPVLCQAHGLTPEQVVAIASNIGGKQALETVQRLLPVLCQAHGLTPEQVVAIASNGGGKQALETVQRLLPVLCQAHGLTPEQVVAIASNGGGKQALETVQRLLPVLCQAHGLTPEQVVAIASHDGGKQALETVQRLLPVLCQAHGLTPEQVVAIASHDGGKQALETVQRLLPVLCQAHGLTPEQVVAIASNIGGKQALETVQRLLPVLCQAHGLTPEQVVAIASNGGGKQALETVQRLLPVLCQAHGLTPEQVVAIASNGGGKQALETVQRLLPVLCQAHGLTPEQVVAIASHDGGKQALETVQRLLPVLCQAHGLTPEQVVAIASHDGGKQALETVQRLLPVLCQAHGLTPEQVVAIASNIGGKQALETVQRLLPVLCQAHGLTPEQVVAIASNGGGRPALESIVAQLSRPDPALAALTNDHLVALACLGGRPALDAVKKGLPHAPALIKRTNRRIPERTSHRVAKGGRADPAFLYKVVSSSSFEFMVSKGEELFTGVVPILVELDGDVNDHKFSVRGEGEGDATNGKLTLKFICTTGKLPVPWPTLVTTFGYGVACFSRYPDHMKQHDFFKSAMPEGYVQERTISFKDDGTYKTRAEVKFEGDTLVNRIELKGIDFKEDGNILGHKLEYNFNSHNVYITADKQKNGIKANFKIRHNVEDGSVQLADHYQQNTPIGDGPVLLPDNHYLSHQSKLSKDPNEKRDHMVLLEFVTAAGITHGMDELYKVDMDSATHIKFSKRDEDGKELAGATMELRDSSGKTISTWISDGQVKDFYLYPGKYTFVETAAPDGYEVATAITFTVNEQGQVTVNGKATKGDAHIGS

SEQ ID NO: 67 - protein, 4116 aa, synthetic construct
GCGAAUUAAUUCGAGCUCGGUACCCAGCUUGCUUGUUCUUUUUGCAGAAGCUCAGAAUAAACGCUCAACUUUGGCAGAUCAAUUCCCCGGUGCUAGCAUGGGUUCCGCCCACAUCGUGAUGGUGGACGCCUACAAGCCGACGAAGACCGGUACAAGUUUGUACAAAAAAGCAGGCUCCGCGGCCGCCCCCUUCACCAUGGUAGAUUUGAGAACUUUGGGAUAUUCACAGCAGCAGCAGGAAAAGAUCAAGCCCAAAGUGAGGUCGACAGUCGCGCAGCAUCACGAAGCGCUGGUGGGUCAUGGGUUUACACAUGCCCACAUCGUAGCCUUGUCGCAGCACCCUGCAGCCCUUGGCACGGUCGCCGUCAAGUACCAGGACAUGAUUGCGGCGUUGCCGGAAGCCACACAUGAGGCGAUCGUCGGUGUGGGGAAACAGUGGAGCGGAGCCCGAGCGCUUGAGGCCCUGUUGACGGUCGCGGGAGAGCUGAGAGGGCCUCCCCUUCAGCUGGACACGGGCCAGUUGCUGAAGAUCGCGAAGCGGGGAGGAGUCACGGCGGUCGAGGCGGUGCACGCGUGGCGCAAUGCGCUCACGGGAGCACCCCUCAACCUGACCCCAGAGCAGGUCGUGGCAAUUGCGAGCCAUGACGGGGGAAAGCAGGCACUCGAAACCGUCCAGAGGUUGCUGCCUGUGCUGUGCCAAGCGCACGGACUUACGCCAGAGCAGGUCGUGGCAAUUGCGAGCCAUGACGGGGGAAAGCAGGCACUCGAAACCGUCCAGAGGUUGCUGCCUGUGCUGUGCCAAGCGCACGGACUAACCCCAGAGCAGGUCGUGGCAAUUGCGAGCAACAUCGGGGGAAAGCAGGCACUCGAAACCGUCCAGAGGUUGCUGCCUGUGCUGUGCCAAGCGCACGGGUUGACCCCAGAGCAGGUCGUGGCAAUUGCGAGCAACGGAGGGGGAAAGCAGGCACUCGAAACCGUCCAGAGGUUGCUGCCUGUGCUGUGCCAAGCGCACGGGUUGACCCCAGAGCAGGUCGUGGCAAUUGCGAGCAACGGAGGGGGAAAGCAGGCACUCGAAACCGUCCAGAGGUUGCUGCCUGUGCUGUGCCAAGCGCACGGACUGACACCAGAGCAGGUCGUGGCAAUUGCGAGCCAUGACGGGGGAAAGCAGGCACUCGAAACCGUCCAGAGGUUGCUGCCUGUGCUGUGCCAAGCGCACGGACUUACACCCGAACAAGUCGUGGCAAUUGCGAGCCAUGACGGGGGAAAGCAGGCACUCGAAACCGUCCAGAGGUUGCUGCCUGUGCUGUGCCAAGCGCACGGACUAACCCCAGAGCAGGUCGUGGCAAUUGCGAGCAACAUCGGGGGAAAGCAGGCACUCGAAACCGUCCAGAGGUUGCUGCCUGUGCUGUGCCAAGCGCACGGGUUGACCCCAGAGCAGGUCGUGGCAAUUGCGAGCAACGGAGGGGGAAAGCAGGCACUCGAAACCGUCCAGAGGUUGCUGCCUGUGCUGUGCCAAGCGCACGGGUUGACCCCAGAGCAGGUCGUGGCAAUUGCGAGCAACGGAGGGGGAAAGCAGGCACUCGAAACCGUCCAGAGGUUGCUGCCUGUGCUGUGCCAAGCGCACGGACUGACACCAGAGCAGGUCGUGGCAAUUGCGAGCCAUGACGGGGGAAAGCAGGCACUCGAAACCGUCCAGAGGUUGCUGCCUGUGCUGUGCCAAGCGCACGGACUUACACCCGAACAAGUCGUGGCAAUUGCGAGCCAUGACGGGGGAAAGCAGGCACUCGAAACCGUCCAGAGGUUGCUGCCUGUGCUGUGCCAAGCGCACGGCCUCACCCCAGAGCAGGUCGUGGCAAUUGCGAGCAACAUCGGGGGAAAGCAGGCACUCGAAACCGUCCAGAGGUUGCUGCCUGUGCUGUGCCAAGCGCACGGACUUACGCCAGAGCAGGUCGUGGCAAUUGCGAGCAACGGAGGGGGAAAGCAGGCACUCGAAACCGUCCAGAGGUUGCUGCCUGUGCUGUGCCAAGCGCACGGACUAACCCCAGAGCAGGUCGUGGCAAUUGCGAGCAACGGAGGGGGAAAGCAGGCACUCGAAACCGUCCAGAGGUUGCUGCCUGUGCUGUGCCAAGCGCACGGGUUGACCCCAGAGCAGGUCGUGGCAAUUGCGAGCCAUGACGGGGGAAAGCAGGCACUCGAAACCGUCCAGAGGUUGCUGCCUGUGCUGUGCCAAGCGCACGGCCUGACCCCAGAGCAGGUCGUGGCAAUUGCGAGCCAUGACGGGGGAAAGCAGGCACUCGAAACCGUCCAGAGGUUGCUGCCUGUGCUGUGCCAAGCGCACGGACUGACACCAGAGCAGGUCGUGGCAAUUGCGAGCAACAUCGGGGGAAAGCAGGCACUCGAAACCGUCCAGAGGUUGCUGCCUGUGCUGUGCCAAGCGCACGGACUCACGCCUGAGCAGGUAGUGGCUAUUGCAUCCAACGGAGGGGGCAGACCCGCACUGGAGUCAAUCGUGGCCCAGCUUUCGAGGCCGGACCCCGCGCUGGCCGCACUCACUAAUGAUCAUCUUGUAGCGCUGGCCUGCCUCGGCGGACGACCCGCCUUGGAUGCGGUGAAGAAGGGGCUCCCGCACGCGCCUGCAUUGAUUAAGCGGACCAACAGAAGGAUUCCCGAGAGGACAUCACAUCGAGUGGCAAAGGGUGGGCGCGCCGACCCAGCUUUCUUGUACAAAGUGGUCCAUUGUGCCCAGCCACCCCCAAAAGCCCUCAGGCGAGAGCUGCCUGAGGAGGCAGCCGCUGAGGAGGAAAGGAGAAAGAUUGAAGUUCCAAGUGAGAUUGAGGUCCCGAGGGAGGCCCUGGAGCCCAGUGUUCCCCUUAUGGUGUCUUUAGAGAUCUCCCUAGAGGCAGCUGAAGAGGAGAAGUCCCGCAUCAGCCUCAUCCCACCAGAAGAACGGUGGGCCUGGCCUGAGGUGGAGGCGCCAGAAGCUCCUGCAUUGCCCGUGGUGCCUGAACUCCCUGAGGUGCCCAUGGAGAUGCCUUUGGUGCUGCCCCCAGAGCUCGAGCUGCUCAGAAUGGUGAGCAAGGGCGAGGAGGAUAACAUGGCCAUCAUCAAGGAGUUCAUGCGCUUCAAGGUGCACAUGGAGGGCUCCGUGAACGGCCACGAGUUCGAGAUCGAGGGCGAGGGCGAGGGCCGCCCCUACGAGGGCACCCAGACCGCCAAGCUGAAGGUGACCAAGGGUGGCCCCCUGCCCUUCGCCUGGGACAUCCUGUCCCCUCAGUUCAUGUACGGCUCCAAGGCCUACGUGAAGCACCCCGCCGACAUCCCCGACUACUUGAAGCUGUCCUUCCCCGAGGGCUUCAAGUGGGAGCGCGUGAUGAACUUCGAGGACGGCGGCGUGGUGACCGUGACCCAGGACUCCUCCCUGCAGGACGGCGAGUUCAUCUACAAGGUGAAGCUGCGCGGCACCAACUUCCCCUCCGACGGCCCCGUAAUGCAGAAGAAGACCAUGGGCUGGGAGGCCUCCUCCGAGCGGAUGUACCCCGAGGACGGCGCCCUGAAGGGCGAGAUCAAGCAGAGGCUGAAGCUGAAGGACGGCGGCCACUACGACGCUGAGGUCAAGACCACCUACAAGGCCAAGAAGCCCGUGCAGCUGCCCGGCGCCUACAACGUCAACAUCAAGUUGGACAUCACCUCCCACAACGAGGACUACACCAUCGUGGAACAGUACGAACGCGCCGAGGGCCGCCACUCCACCGGCGGCAUGGACGAGCUGUACAAGAAAAGCUUAGGUUCCGCCCAUAUAGUUAUGGUGGACGCCUAUAAACCCACUAAGAGUCGACGGCCCGGGAUCCUGUACAAGUAAAGCGGCCGCUCUAGAUAAAUGAUAGCUUGAUCUGGUUACCACUAAACCAGCCUCAAGAACACCCGAAUGGAGUCUCUAAGCUACAUAAUACCAACUUACACUUUACAAAAUGUUGUCCCCCAAAAUGUAGCCAUUCGUAUCUGCUCCUAAUAAAAAGAAAGUUUCUUCACAUUCUAAAAAAAAAAAAAAAAAAAAAAAAAAAAAAAAAACCCCCCCCCCCCCCCCCUGCAGGCGCGCCGCCGGCGAUUUAAAUUAAU

SEQ ID NO: 68 - protein, 1253 aa, synthetic construct
MGSAHIVMVDAYKPTKTGTSLYKKAGSAAAPFTMVDLRTLGYSQQQQEKIKPKVRSTVAQHHEALVGHGFTHAHIVALSQHPAALGTVAVKYQDMIAALPEATHEAIVGVGKQWSGARALEALLTVAGELRGPPLQLDTGQLLKIAKRGGVTAVEAVHAWRNALTGAPLNLTPEQVVAIASHDGGKQALETVQRLLPVLCQAHGLTPEQVVAIASHDGGKQALETVQRLLPVLCQAHGLTPEQVVAIASNIGGKQALETVQRLLPVLCQAHGLTPEQVVAIASNGGGKQALETVQRLLPVLCQAHGLTPEQVVAIASNGGGKQALETVQRLLPVLCQAHGLTPEQVVAIASHDGGKQALETVQRLLPVLCQAHGLTPEQVVAIASHDGGKQALETVQRLLPVLCQAHGLTPEQVVAIASNIGGKQALETVQRLLPVLCQAHGLTPEQVVAIASNGGGKQALETVQRLLPVLCQAHGLTPEQVVAIASNGGGKQALETVQRLLPVLCQAHGLTPEQVVAIASHDGGKQALETVQRLLPVLCQAHGLTPEQVVAIASHDGGKQALETVQRLLPVLCQAHGLTPEQVVAIASNIGGKQALETVQRLLPVLCQAHGLTPEQVVAIASNGGGKQALETVQRLLPVLCQAHGLTPEQVVAIASNGGGKQALETVQRLLPVLCQAHGLTPEQVVAIASHDGGKQALETVQRLLPVLCQAHGLTPEQVVAIASHDGGKQALETVQRLLPVLCQAHGLTPEQVVAIASNIGGKQALETVQRLLPVLCQAHGLTPEQVVAIASNGGGRPALESIVAQLSRPDPALAALTNDHLVALACLGGRPALDAVKKGLPHAPALIKRTNRRIPERTSHRVAKGGRADPAFLYKVVHCAQPPPKALRRELPEEAAAEEERRKIEVPSEIEVPREALEPSVPLMVSLEISLEAAEEEKSRISLIPPEERWAWPEVEAPEAPALPVVPELPEVPMEMPLVLPPELELLRMVSKGEEDNMAIIKEFMRFKVHMEGSVNGHEFEIEGEGEGRPYEGTQTAKLKVTKGGPLPFAWDILSPQFMYGSKAYVKHPADIPDYLKLSFPEGFKWERVMNFEDGGVVTVTQDSSLQDGEFIYKVKLRGTNFPSDGPVMQKKTMGWEASSERMYPEDGALKGEIKQRLKLKDGGHYDAEVKTTYKAKKPVQLPGAYNVNIKLDITSHNEDYTIVEQYERAEGRHSTGGMDELYKKSLGSAHIVMVDAYKPTKSRRPGILYK

SEQ ID NO: 69 - RNA, 4586 nt, synthetic construct
  source 1..4586: mol_type = other RNA
gcgaattaattcgagctcggtacccagcttgcttgttctttttgcagaagctcagaataaacgctcaactttggcagatcaattccccggtgctagcatggatagtgctacccatattaaattctcaaaacgtgatgaggacggcaaagagttagctggtgcaactatggagttgcgtgattcatctggtaaaactattagtacatggatttcagatggacaagtgaaagatttctacctgtatccaggaaaatatacatttgtcgaaaccgcagcaccagacggttatgaggtagcaactgctattacctttacagttaatgagcaaggtcaggttactgtaaatggcaaagcaactaaaggtgacgctcatattggatccaccggtacaagtttgtacaaaaaagcaggctccgcggccgcccccttcaccatggtagatttgagaactttgggatattcacagcagcagcaggaaaagatcaagcccaaagtgaggtcgacagtcgcgcagcatcacgaagcgctggtgggtcatgggtttacacatgcccacatcgtagccttgtcgcagcaccctgcagcccttggcacggtcgccgtcaagtaccaggacatgattgcggcgttgccggaagccacacatgaggcgatcgtcggtgtggggaaacagtggagcggagcccgagcgcttgaggccctgttgacggtcgcgggagagctgagagggcctccccttcagctggacacgggccagttgctgaagatcgcgaagcggggaggagtcacggcggtcgaggcggtgcacgcgtggcgcaatgcgctcacgggagcacccctcaacctgaccccagagcaggtcgtggcaattgcgagccatgacgggggaaagcaggcactcgaaaccgtccagaggttgctgcctgtgctgtgccaagcgcacggacttacgccagagcaggtcgtggcaattgcgagccatgacgggggaaagcaggcactcgaaaccgtccagaggttgctgcctgtgctgtgccaagcgcacggactaaccccagagcaggtcgtggcaattgcgagcaacatcgggggaaagcaggcactcgaaaccgtccagaggttgctgcctgtgctgtgccaagcgcacgggttgaccccagagcaggtcgtggcaattgcgagcaacggagggggaaagcaggcactcgaaaccgtccagaggttgctgcctgtgctgtgccaagcgcacgggttgaccccagagcaggtcgtggcaattgcgagcaacggagggggaaagcaggcactcgaaaccgtccagaggttgctgcctgtgctgtgccaagcgcacggactgacaccagagcaggtcgtggcaattgcgagccatgacgggggaaagcaggcactcgaaaccgtccagaggttgctgcctgtgctgtgccaagcgcacggacttacacccgaacaagtcgtggcaattgcgagccatgacgggggaaagcaggcactcgaaaccgtccagaggttgctgcctgtgctgtgccaagcgcacggactaaccccagagcaggtcgtggcaattgcgagcaacatcgggggaaagcaggcactcgaaaccgtccagaggttgctgcctgtgctgtgccaagcgcacgggttgaccccagagcaggtcgtggcaattgcgagcaacggagggggaaagcaggcactcgaaaccgtccagaggttgctgcctgtgctgtgccaagcgcacgggttgaccccagagcaggtcgtggcaattgcgagcaacggagggggaaagcaggcactcgaaaccgtccagaggttgctgcctgtgctgtgccaagcgcacggactgacaccagagcaggtcgtggcaattgcgagccatgacgggggaaagcaggcactcgaaaccgtccagaggttgctgcctgtgctgtgccaagcgcacggacttacacccgaacaagtcgtggcaattgcgagccatgacgggggaaagcaggcactcgaaaccgtccagaggttgctgcctgtgctgtgccaagcgcacggcctcaccccagagcaggtcgtggcaattgcgagcaacatcgggggaaagcaggcactcgaaaccgtccagaggttgctgcctgtgctgtgccaagcgcacggacttacgccagagcaggtcgtggcaattgcgagcaacggagggggaaagcaggcactcgaaaccgtccagaggttgctgcctgtgctgtgccaagcgcacggactaaccccagagcaggtcgtggcaattgcgagcaacggagggggaaagcaggcactcgaaaccgtccagaggttgctgcctgtgctgtgccaagcgcacgggttgaccccagagcaggtcgtggcaattgcgagccatgacgggggaaagcaggcactcgaaaccgtccagaggttgctgcctgtgctgtgccaagcgcacggcctgaccccagagcaggtcgtggcaattgcgagccatgacgggggaaagcaggcactcgaaaccgtccagaggttgctgcctgtgctgtgccaagcgcacggactgacaccagagcaggtcgtggcaattgcgagcaacatcgggggaaagcaggcactcgaaaccgtccagaggttgctgcctgtgctgtgccaagcgcacggactcacgcctgagcaggtagtggctattgcatccaacggagggggcagacccgcactggagtcaatcgtggcccagctttcgaggccggaccccgcgctggccgcactcactaatgatcatcttgtagcgctggcctgcctcggcggacgacccgccttggatgcggtgaagaaggggctcccgcacgcgcctgcattgattaagcggaccaacagaaggattcccgagaggacatcacatcgagtggcaaagggtgggcgcgccgacccagctttcttgtacaaagtggtctcgagctcacattgtgcccagccacccccaaaagccctcaggcgagagctgcctgaggaggcagccgctgaggaggaaaggagaaagattgaagttccaagtgagattgaggtcccgagggaggccctggagcccagtgttccccttatggtgtctttagagatctccctagaggcagctgaagaggagaagtcccgcatcagcctcatcccaccagaagaacggtgggcctggcctgaggtggaggcgccagaagctcctgcattgcccgtggtgcctgaactccctgaggtgcccatggagatgcctttggtgctgcccccagagctcgagctgctcatcgaattcatggtgagcaagggcgaggagctgttcaccggggtggtgcccatcctggtcgagctggacggcgacgtaaacgaccacaagttcagcgtccgcggcgagggcgagggcgatgccaccaacggcaagctgaccctgaagttcatctgcaccaccggcaagctgcccgtgccctggcccaccctcgtgaccaccttcggctacggcgtggcctgcttcagccgctaccccgaccacatgaagcagcacgacttcttcaagtccgccatgcccgaaggctacgtccaggagcgcaccatctctttcaaggacgacggtacctacaagacccgcgccgaggtgaagttcgagggcgacaccctggtgaaccgcatcgagctgaagggcatcgacttcaaggaggacggcaacatcctggggcacaagctggagtacaacttcaacagccacaacgtctatatcacggccgacaagcagaagaacggcatcaaggctaacttcaagatccgccacaacgttgaggacggcagcgtgcagctcgccgaccactaccagcagaacacccccatcggcgacggccccgtgctgctgcccgacaaccactacctgagccatcagtccaagctgagcaaagaccccaacgagaagcgcgatcacatggtcctgctggagttcgtgaccgccgccgggattacacatggcatggacgagctgtacaaggtcgacatggatagtgctacccatattaaattctcaaaacgtgatgaggacggcaaagagttagctggtgcaactatggagttgcgtgattcatctggtaaaactattagtacatggatttcagatggacaagtgaaagatttctacctgtatccaggaaaatatacatttgtcgaaaccgcagcaccagacggttatgaggtagcaactgctattacctttacagttaatgagcaaggtcaggttactgtaaatggcaaagcaactaaaggtgacgctcatattggatcctaagcggccgctctagataaatgatagcttgatctggttaccactaaaccagcctcaagaacacccgaatggagtctctaagctacataataccaacttacactttacaaaatgttgtcccccaaaatgtagccattcgtatctgctcctaataaaaagaaagtttcttcacattctaaaaaaaaaaaaaaaaaaaaaaaaaaaaaaaaaaccccccccccccccccctgcaggcgcgccgccggcgatttaaattaat

SEQ ID NO: 70 - protein, 1410 aa, synthetic construct
MDSATHIKFSKRDEDGKELAGATMELRDSSGKTISTWISDGQVKDFYLYPGKYTFVETAAPDGYEVATAITFTVNEQGQVTVNGKATKGDAHIGSTGTSLYKKAGSAAAPFTMVDLRTLGYSQQQQEKIKPKVRSTVAQHHEALVGHGFTHAHIVALSQHPAALGTVAVKYQDMIAALPEATHEAIVGVGKQWSGARALEALLTVAGELRGPPLQLDTGQLLKIAKRGGVTAVEAVHAWRNALTGAPLNLTPEQVVAIASHDGGKQALETVQRLLPVLCQAHGLTPEQVVAIASHDGGKQALETVQRLLPVLCQAHGLTPEQVVAIASNIGGKQALETVQRLLPVLCQAHGLTPEQVVAIASNGGGKQALETVQRLLPVLCQAHGLTPEQVVAIASNGGGKQALETVQRLLPVLCQAHGLTPEQVVAIASHDGGKQALETVQRLLPVLCQAHGLTPEQVVAIASHDGGKQALETVQRLLPVLCQAHGLTPEQVVAIASNIGGKQALETVQRLLPVLCQAHGLTPEQVVAIASNGGGKQALETVQRLLPVLCQAHGLTPEQVVAIASNGGGKQALETVQRLLPVLCQAHGLTPEQVVAIASHDGGKQALETVQRLLPVLCQAHGLTPEQVVAIASHDGGKQALETVQRLLPVLCQAHGLTPEQVVAIASNIGGKQALETVQRLLPVLCQAHGLTPEQVVAIASNGGGKQALETVQRLLPVLCQAHGLTPEQVVAIASNGGGKQALETVQRLLPVLCQAHGLTPEQVVAIASHDGGKQALETVQRLLPVLCQAHGLTPEQVVAIASHDGGKQALETVQRLLPVLCQAHGLTPEQVVAIASNIGGKQALETVQRLLPVLCQAHGLTPEQVVAIASNGGGRPALESIVAQLSRPDPALAALTNDHLVALACLGGRPALDAVKKGLPHAPALIKRTNRRIPERTSHRVAKGGRADPAFLYKVVSSSHCAQPPPKALRRELPEEAAAEEERRKIEVPSEIEVPREALEPSVPLMVSLEISLEAAEEEKSRISLIPPEERWAWPEVEAPEAPALPVVPELPEVPMEMPLVLPPELELLIEFMVSKGEELFTGVVPILVELDGDVNDHKFSVRGEGEGDATNGKLTLKFICTTGKLPVPWPTLVTTFGYGVACFSRYPDHMKQHDFFKSAMPEGYVQERTISFKDDGTYKTRAEVKFEGDTLVNRIELKGIDFKEDGNILGHKLEYNFNSHNVYITADKQKNGIKANFKIRHNVEDGSVQLADHYQQNTPIGDGPVLLPDNHYLSHQSKLSKDPNEKRDHMVLLEFVTAAGITHGMDELYKVDMDSATHIKFSKRDEDGKELAGATMELRDSSGKTISTWISDGQVKDFYLYPGKYTFVETAAPDGYEVATAITFTVNEQGQVTVNGKATKGDAHIGS

SEQ ID NO: 71 - RNA, 2133 nt, synthetic construct; identical to SEQ ID NO: 9
  source 1..2133: mol_type = other RNA

SEQ ID NO: 72 - protein, 711 aa, synthetic construct; identical to SEQ ID NO: 10

SEQ ID NO: 73 - RNA, 3614 nt, synthetic construct
  source 1..3614: mol_type = other RNA
gcgaattaattcgagctcggtacccagcttgcttgttctttttgcagaagctcagaataaacgctcaactttggcagatcaattccccggtgctagcacaagtttgtacaaaaaagcaggctccgcggccgcccccttcaccatggctactcttatctttgttgataaggataatgaagaacccggccgccgtttggcatctaaggatgggttgaagctgggcactggtgtcaaggccttagatgggaaattgcaggtttcaacgcctcgagtcggcaaagtgttcaatgctccagccgtgcctaaagccagcagaaaggctttggggacagtcaacagagttgccgaaaagcctatgaagactggcaaacccctccaaccaaaacagccgaccttgactgggaaaaagatcaccgagaagtctactaagacacaaagttctgttaagggtgggcgcgccgacccagctttcttgtacaaagtggtaagcttcgaattcatggtgagcaagggcgaggagctgttcaccggggtggtgcccatcctggtcgagctggacggcgacgtaaacgaccacaagttcagcgtccgcggcgagggcgagggcgatgccaccaacggcaagctgaccctgaagttcatctgcaccaccggcaagctgcccgtgccctggcccaccctcgtgaccaccttcggctacggcgtggcctgcttcagccgctaccccgaccacatgaagcagcacgacttcttcaagtccgccatgcccgaaggctacgtccaggagcgcaccatctctttcaaggacgacggtacctacaagacccgcgccgaggtgaagttcgagggcgacaccctggtgaaccgcatcgagctgaagggcatcgacttcaaggaggacggcaacatcctggggcacaagctggagtacaacttcaacagccacaacgtctatatcacggccgacaagcagaagaacggcatcaaggctaacttcaagatccgccacaacgttgaggacggcagcgtgcagctcgccgaccactaccagcagaacacccccatcggcgacggccccgtgctgctgcccgacaaccactacctgagccatcagtccaagctgagcaaagaccccaacgagaagcgcgatcacatggtcctgctggagttcgtgaccgccgccgggattacacatggcatggacgagctgtacaaggtcgacatgcaggtggatctacgcacgctcggctacagtcagcagcagcaagagaagatcaaaccgaaggtgcgttcgacagtggcgcagcaccacgaggcactggtgggccatgggtttacacacgcgcacatcgttgcgctcagccaacacccggcagcgttagggaccgtcgctgtcacgtatcagcacataatcacggcgttgccagaggcgacacacgaagacatcgttggcgtcggcaaacagtggtccggcgcacgcgccctggaggccttgctcacggatgcgggggagttgagaggtccgccgttacagttggacacaggccaacttgtgaagattgcaaaacgtggcggcgtgaccgcaatggaggcagtgcatgcatcgcgcaatgcactgacgggtgcccccctgaacctgaccccggaccaagtggtggctatcgccagcaacggtggcggcaagcaagcgctcgaaacggtgcagcggctgttgccggtgctgtgccaggaccatggcctgaccccggaccaagtggtggctatcgccagcaacaagggcggcaagcaagcgctcgaaacggtgcagcggctgttgccggtgctgtgccaggaccatggcctgactccggaccaagtggtggctatcgccagccacgatggcggcaagcaagcgctcgaaacggtgcagcggctgttgccggtgctgtgccaggaccatggcctgactccggaccaagtggtggctatcgccagccacgatggcggcaagcaagcgctcgaaacggtgcagcggctgttgccggtgctgtgccaggaccatggcctgaccccggaccaagtggtggctatcgccagcaacattggcggcaagcaagcgctcgaaacggtgcagcggctgttgccggtgctgtgccaggaccatggcctgaccccggaccaagtggtggctatcgccagcaacggtggcggcaagcaagcgctcgaaacggtgcagcggctgttgccggtgctgtgccaggaccatggcctgaccccggaccaagtggtggctatcgccagcaacattggcggcaagcaagcgctcgaaacggtgcagcggctgttgccggtgctgtgccaggaccatggcctgaccccggaccaagtggtggctatcgccagcaacggtggcggcaagcaagcgctcgaaacggtgcagcggctgttgccggtgctgtgccaggaccatggcctgaccccggaccaagtggtggctatcgccagcaacggtggcggcaagcaagcgctcgaaacggtgcagcggctgttgccggtgctgtgccaggaccatggcctgactccggaccaagtggtggctatcgccagccacgatggcggcaagcaagcgctcgaaacggtgcagcggctgttgccggtgctgtgccaggaccatggcctgaccccggaccaagtggtggctatcgccagccacgatggcggcaagcaagcgctcgaaacggtgcagcggctgttgccggtgctgtgccaggaccatggcctgaccccggaccaagtggtggctatcgccagcaacattggcggcaagcaagcgctcgaaacggtgcagcggctgttgccggtgctgtgccaggaccatggcctgactccggaccaagtggtggctatcgccagccacgatggcggcaagcaagcgctcgaaacggtgcagcggctgttgccggtgctgtgccaggaccatggcctgaccccggaccaagtggtggctatcgccagcaacaagggcggcaagcaagcgctcgaaacggtgcagcggctgttgccggtgctgtgccaggaccatggcctgaccccggaccaagtggtggctatcgccagcaacggtggcggcaagcaagcgctcgaaagcattgtggcccagctgagccggcctgatccggcgttggccgcgttgaccaacgaccacctcgtcgccttggcctgcctcggcggacgtcctgccatggatgcagtgaaaaagggattgccgcacgcgccggaattgatcagaagagtcaatcgccgtattggcgaacgcacgtcccatcgcgttgcgggatccactggaggcggaggtggctccggcaccgcctcctcctaagcggccgctctagataaatgatagcttgatctggttaccactaaaccagcctcaagaacacccgaatggagtctctaagctacataataccaacttacactttacaaaatgttgtcccccaaaatgtagccattcgtatctgctcctaataaaaagaaagtttcttcacattctaaaaaaaaaaaaaaaaaaaaaaaaaaaaaaaaaaccccccccccccccccctgcaggcgcgccgccggcgatttaaattaat

SEQ ID NO: 74 - protein, 1071 aa, synthetic construct
MATLIFVDKDNEEPGRRLASKDGLKLGTGVKALDGKLQVSTPRVGKVFNAPAVPKASRKALGTVNRVAEKPMKTGKPLQPKQPTLTGKKITEKSTKTQSSVKGGRADPAFLYKVVSFEFMVSKGEELFTGVVPILVELDGDVNDHKFSVRGEGEGDATNGKLTLKFICTTGKLPVPWPTLVTTFGYGVACFSRYPDHMKQHDFFKSAMPEGYVQERTISFKDDGTYKTRAEVKFEGDTLVNRIELKGIDFKEDGNILGHKLEYNFNSHNVYITADKQKNGIKANFKIRHNVEDGSVQLADHYQQNTPIGDGPVLLPDNHYLSHQSKLSKDPNEKRDHMVLLEFVTAAGITHGMDELYKVDMQVDLRTLGYSQQQQEKIKPKVRSTVAQHHEALVGHGFTHAHIVALSQHPAALGTVAVTYQHIITALPEATHEDIVGVGKQWSGARALEALLTDAGELRGPPLQLDTGQLVKIAKRGGVTAMEAVHASRNALTGAPLNLTPDQVVAIASNGGGKQALETVQRLLPVLCQDHGLTPDQVVAIASNKGGKQALETVQRLLPVLCQDHGLTPDQVVAIASHDGGKQALETVQRLLPVLCQDHGLTPDQVVAIASHDGGKQALETVQRLLPVLCQDHGLTPDQVVAIASNIGGKQALETVQRLLPVLCQDHGLTPDQVVAIASNGGGKQALETVQRLLPVLCQDHGLTPDQVVAIASNIGGKQALETVQRLLPVLCQDHGLTPDQVVAIASNGGGKQALETVQRLLPVLCQDHGLTPDQVVAIASNGGGKQALETVQRLLPVLCQDHGLTPDQVVAIASHDGGKQALETVQRLLPVLCQDHGLTPDQVVAIASHDGGKQALETVQRLLPVLCQDHGLTPDQVVAIASNIGGKQALETVQRLLPVLCQDHGLTPDQVVAIASHDGGKQALETVQRLLPVLCQDHGLTPDQVVAIASNKGGKQALETVQRLLPVLCQDHGLTPDQVVAIASNGGGKQALESIVAQLSRPDPALAALTNDHLVALACLGGRPAMDAVKKGLPHAPELIRRVNRRIGERTSHRVAGSTGGGGGSGTASS

SEQ ID NO: 75 - RNA, 3548 nt, synthetic construct
  source 1..3548: mol_type = other RNA
gcgaattaattcgagctcggtacccagcttgcttgttctttttgcagaagctcagaataaacgctcaactttggcagatcaattccccggtgctagcacaagtttgtacaaaaaagcaggctccgcggccgcccccttcaccatggcgctcagggtcactaggaacacgaaaattaacgcagaaaataaggccaaggtcagtatggcaggcgccaagcgtgtgcctgtgacagttactgctgcttccaagcccgggctgagaccgagaactgctcttggagacattggtaataaagtcagcgaagagctacaggcaagagtgcctctgaaaagggaagcaaaaacgctaggtactggaaaaggtactgttaaagccctaaagggtgggcgcgccgacccagctttcttgtacaaagtggtaagcttcgaattcatggtgagcaagggcgaggagctgttcaccggggtggtgcccatcctggtcgagctggacggcgacgtaaacgaccacaagttcagcgtccgcggcgagggcgagggcgatgccaccaacggcaagctgaccctgaagttcatctgcaccaccggcaagctgcccgtgccctggcccaccctcgtgaccaccttcggctacggcgtggcctgcttcagccgctaccccgaccacatgaagcagcacgacttcttcaagtccgccatgcccgaaggctacgtccaggagcgcaccatctctttcaaggacgacggtacctacaagacccgcgccgaggtgaagttcgagggcgacaccctggtgaaccgcatcgagctgaagggcatcgacttcaaggaggacggcaacatcctggggcacaagctggagtacaacttcaacagccacaacgtctatatcacggccgacaagcagaagaacggcatcaaggctaacttcaagatccgccacaacgttgaggacggcagcgtgcagctcgccgaccactaccagcagaacacccccatcggcgacggccccgtgctgctgcccgacaaccactacctgagccatcagtccaagctgagcaaagaccccaacgagaagcgcgatcacatggtcctgctggagttcgtgaccgccgccgggattacacatggcatggacgagctgtacaaggtcgacatgcaggtggatctacgcacgctcggctacagtcagcagcagcaagagaagatcaaaccgaaggtgcgttcgacagtggcgcagcaccacgaggcactggtgggccatgggtttacacacgcgcacatcgttgcgctcagccaacacccggcagcgttagggaccgtcgctgtcacgtatcagcacataatcacggcgttgccagaggcgacacacgaagacatcgttggcgtcggcaaacagtggtccggcgcacgcgccctggaggccttgctcacggatgcgggggagttgagaggtccgccgttacagttggacacaggccaacttgtgaagattgcaaaacgtggcggcgtgaccgcaatggaggcagtgcatgcatcgcgcaatgcactgacgggtgcccccctgaacctgaccccggaccaagtggtggctatcgccagcaacggtggcggcaagcaagcgctcgaaacggtgcagcggctgttgccggtgctgtgccaggaccatggcctgaccccggaccaagtggtggctatcgccagcaacaagggcggcaagcaagcgctcgaaacggtgcagcggctgttgccggtgctgtgccaggaccatggcctgactccggaccaagtggtggctatcgccagccacgatggcggcaagcaagcgctcgaaacggtgcagcggctgttgccggtgctgtgccaggaccatggcctgactccggaccaagtggtggctatcgccagccacgatggcggcaagcaagcgctcgaaacggtgcagcggctgttgccggtgctgtgccaggaccatggcctgaccccggaccaagtggtggctatcgccagcaacattggcggcaagcaagcgctcgaaacggtgcagcggctgttgccggtgctgtgccaggaccatggcctgaccccggaccaagtggtggctatcgccagcaacggtggcggcaagcaagcgctcgaaacggtgcagcggctgttgccggtgctgtgccaggaccatggcctgaccccggaccaagtggtggctatcgccagcaacattggcggcaagcaagcgctcgaaacggtgcagcggctgttgccggtgctgtgccaggaccatggcctgaccccggaccaagtggtggctatcgccagcaacggtggcggcaagcaagcgctcgaaacggtgcagcggctgttgccggtgctgtgccaggaccatggcctgaccccggaccaagtggtggctatcgccagcaacggtggcggcaagcaagcgctcgaaacggtgcagcggctgttgccggtgctgtgccaggaccatggcctgactccggaccaagtggtggctatcgccagccacgatggcggcaagcaagcgctcgaaacggtgcagcggctgttgccggtgctgtgccaggaccatggcctgaccccggaccaagtggtggctatcgccagccacgatggcggcaagcaagcgctcgaaacggtgcagcggctgttgccggtgctgtgccaggaccatggcctgaccccggaccaagtggtggctatcgccagcaacattggcggcaagcaagcgctcgaaacggtgcagcggctgttgccggtgctgtgccaggaccatggcctgactccggaccaagtggtggctatcgccagccacgatggcggcaagcaagcgctcgaaacggtgcagcggctgttgccggtgctgtgccaggaccatggcctgaccccggaccaagtggtggctatcgccagcaacaagggcggcaagcaagcgctcgaaacggtgcagcggctgttgccggtgctgtgccaggaccatggcctgaccccggaccaagtggtggctatcgccagcaacggtggcggcaagcaagcgctcgaaagcattgtggcccagctgagccggcctgatccggcgttggccgcgttgaccaacgaccacctcgtcgccttggcctgcctcggcggacgtcctgccatggatgcagtgaaaaagggattgccgcacgcgccggaattgatcagaagagtcaatcgccgtattggcgaacgcacgtcccatcgcgttgcgggatccactggaggcggaggtggctccggcaccgcctcctcctaagcggccgctctagataaatgatagcttgatctggttaccactaaaccagcctcaagaacacccgaatggagtctctaagctacataataccaacttacactttacaaaatgttgtcccccaaaatgtagccattcgtatctgctcctaataaaaagaaagtttcttcacattctaaaaaaaaaaaaaaaaaaaaaaaaaaaaaaaaaaccccccccccccccccctgcaggcgcgccgccggcgatttaaattaat

SEQ ID NO: 76 - protein, 1049 aa, synthetic construct
MALRVTRNTKINAENKAKVSMAGAKRVPVTVTAASKPGLRPRTALGDIGNKVSEELQARVPLKREAKTLGTGKGTVKALKGGRADPAFLYKVVSFEFMVSKGEELFTGVVPILVELDGDVNDHKFSVRGEGEGDATNGKLTLKFICTTGKLPVPWPTLVTTFGYGVACFSRYPDHMKQHDFFKSAMPEGYVQERTISFKDDGTYKTRAEVKFEGDTLVNRIELKGIDFKEDGNILGHKLEYNFNSHNVYITADKQKNGIKANFKIRHNVEDGSVQLADHYQQNTPIGDGPVLLPDNHYLSHQSKLSKDPNEKRDHMVLLEFVTAAGITHGMDELYKVDMQVDLRTLGYSQQQQEKIKPKVRSTVAQHHEALVGHGFTHAHIVALSQHPAALGTVAVTYQHIITALPEATHEDIVGVGKQWSGARALEALLTDAGELRGPPLQLDTGQLVKIAKRGGVTAMEAVHASRNALTGAPLNLTPDQVVAIASNGGGKQALETVQRLLPVLCQDHGLTPDQVVAIASNKGGKQALETVQRLLPVLCQDHGLTPDQVVAIASHDGGKQALETVQRLLPVLCQDHGLTPDQVVAIASHDGGKQALETVQRLLPVLCQDHGLTPDQVVAIASNIGGKQALETVQRLLPVLCQDHGLTPDQVVAIASNGGGKQALETVQRLLPVLCQDHGLTPDQVVAIASNIGGKQALETVQRLLPVLCQDHGLTPDQVVAIASNGGGKQALETVQRLLPVLCQDHGLTPDQVVAIASNGGGKQALETVQRLLPVLCQDHGLTPDQVVAIASHDGGKQALETVQRLLPVLCQDHGLTPDQVVAIASHDGGKQALETVQRLLPVLCQDHGLTPDQVVAIASNIGGKQALETVQRLLPVLCQDHGLTPDQVVAIASHDGGKQALETVQRLLPVLCQDHGLTPDQVVAIASNKGGKQALETVQRLLPVLCQDHGLTPDQVVAIASNGGGKQALESIVAQLSRPDPALAALTNDHLVALACLGGRPAMDAVKKGLPHAPELIRRVNRRIGERTSHRVAGSTGGGGGSGTASS

SEQ ID NO: 77 - RNA, 3558 nt, synthetic construct
  source 1..3558: mol_type = other RNA
gcgaattaattcgagctcggtacccagcttgcttgttctttttgcagaagctcagaataaacgctcaactttggcagatcaattccccggtgctagcatgggttccgcccacatcgtgatggtggacgcctacaagccgacgaagaccggtggttccagttctgacaccgaggacgtggtgtgctgcagcatgagctacacctggaccggcaagactacaagtttgtacaaaaaagcaggctccgcggccgcccccttcaccatgcaggtggatctacgcacgctcggctacagtcagcagcagcaagagaagatcaaaccgaaggtgcgttcgacagtggcgcagcaccacgaggcactggtgggccatgggtttacacacgcgcacatcgttgcgctcagccaacacccggcagcgttagggaccgtcgctgtcacgtatcagcacataatcacggcgttgccagaggcgacacacgaagacatcgttggcgtcggcaaacagtggtccggcgcacgcgccctggaggccttgctcacggatgcgggggagttgagaggtccgccgttacagttggacacaggccaacttgtgaagattgcaaaacgtggcggcgtgaccgcaatggaggcagtgcatgcatcgcgcaatgcactgacgggtgcccccctgaacctgaccccggaccaagtggtggctatcgccagcaacggtggcggcaagcaagcgctcgaaacggtgcagcggctgttgccggtgctgtgccaggaccatggcctgaccccggaccaagtggtggctatcgccagcaacaagggcggcaagcaagcgctcgaaacggtgcagcggctgttgccggtgctgtgccaggaccatggcctgactccggaccaagtggtggctatcgccagccacgatggcggcaagcaagcgctcgaaacggtgcagcggctgttgccggtgctgtgccaggaccatggcctgactccggaccaagtggtggctatcgccagccacgatggcggcaagcaagcgctcgaaacggtgcagcggctgttgccggtgctgtgccaggaccatggcctgaccccggaccaagtggtggctatcgccagcaacattggcggcaagcaagcgctcgaaacggtgcagcggctgttgccggtgctgtgccaggaccatggcctgaccccggaccaagtggtggctatcgccagcaacggtggcggcaagcaagcgctcgaaacggtgcagcggctgttgccggtgctgtgccaggaccatggcctgaccccggaccaagtggtggctatcgccagcaacattggcggcaagcaagcgctcgaaacggtgcagcggctgttgccggtgctgtgccaggaccatggcctgaccccggaccaagtggtggctatcgccagcaacggtggcggcaagcaagcgctcgaaacggtgcagcggctgttgccggtgctgtgccaggaccatggcctgaccccggaccaagtggtggctatcgccagcaacggtggcggcaagcaagcgctcgaaacggtgcagcggctgttgccggtgctgtgccaggaccatggcctgactccggaccaagtggtggctatcgccagccacgatggcggcaagcaagcgctcgaaacggtgcagcggctgttgccggtgctgtgccaggaccatggcctgaccccggaccaagtggtggctatcgccagccacgatggcggcaagcaagcgctcgaaacggtgcagcggctgttgccggtgctgtgccaggaccatggcctgaccccggaccaagtggtggctatcgccagcaacattggcggcaagcaagcgctcgaaacggtgcagcggctgttgccggtgctgtgccaggaccatggcctgactccggaccaagtggtggctatcgccagccacgatggcggcaagcaagcgctcgaaacggtgcagcggctgttgccggtgctgtgccaggaccatggcctgaccccggaccaagtggtggctatcgccagcaacaagggcggcaagcaagcgctcgaaacggtgcagcggctgttgccggtgctgtgccaggaccatggcctgaccccggaccaagtggtggctatcgccagcaacggtggcggcaagcaagcgctcgaaagcattgtggcccagctgagccggcctgatccggcgttggccgcgttgaccaacgaccacctcgtcgccttggcctgcctcggcggacgtcctgccatggatgcagtgaaaaagggattgccgcacgcgccggaattgatcagaagagtcaatcgccgtattggcgaacgcacgtcccatcgcgttgcgggatccactggaggcggaggtggctccggcaccgcctcctccaagggtgggcgcgccgacccagctttcttgtacaaagtggttgacactgaggatgtagtatgctgtagcatgagttacacttggacaggcaagggatcaagttcatcctcgagaatggtgagcaagggcgaggaggataacatggccatcatcaaggagttcatgcgcttcaaggtgcacatggagggctccgtgaacggccacgagttcgagatcgagggcgagggcgagggccgcccctacgagggcacccagaccgccaagctgaaggtgaccaagggtggccccctgcccttcgcctgggacatcctgtcccctcagttcatgtacggctccaaggcctacgtgaagcaccccgccgacatccccgactacttgaagctgtccttccccgagggcttcaagtgggagcgcgtgatgaacttcgaggacggcggcgtggtgaccgtgacccaggactcctccctgcaggacggcgagttcatctacaaggtgaagctgcgcggcaccaacttcccctccgacggccccgtaatgcagaagaagaccatgggctgggaggcctcctccgagcggatgtaccccgaggacggcgccctgaagggcgagatcaagcagaggctgaagctgaaggacggcggccactacgacgctgaggtcaagaccacctacaaggccaagaagcccgtgcagctgcccggcgcctacaacgtcaacatcaagttggacatcacctcccacaacgaggactacaccatcgtggaacagtacgaacgcgccgagggccgccactccaccggcggcatggacgagctgtacaagaaaagcttaggttccgcccatatagttatggtggacgcctataaacccactaagagtcgacggcccgggatcctgtacaagtaaagcggccgctctagataaatgatagcttgatctggttaccactaaaccagcctcaagaacacccgaatggagtctctaagctacataataccaacttacactttacaaaatgttgtcccccaaaatgtagccattcgtatctgctcctaataaaaagaaagtttcttcacattctaaaaaaaaaaaaaaaaaaaaaaaaaaaaaaaaaaccccccccccccccccctgcaggcgcgccgccggcgatttaaattaat

SEQ ID NO: 78 - protein, 1067 aa, synthetic construct
MGSAHIVMVDAYKPTKTGGSSSDTEDVVCCSMSYTWTGKTTSLYKKAGSAAAPFTMQVDLRTLGYSQQQQEKIKPKVRSTVAQHHEALVGHGFTHAHIVALSQHPAALGTVAVTYQHIITALPEATHEDIVGVGKQWSGARALEALLTDAGELRGPPLQLDTGQLVKIAKRGGVTAMEAVHASRNALTGAPLNLTPDQVVAIASNGGGKQALETVQRLLPVLCQDHGLTPDQVVAIASNKGGKQALETVQRLLPVLCQDHGLTPDQVVAIASHDGGKQALETVQRLLPVLCQDHGLTPDQVVAIASHDGGKQALETVQRLLPVLCQDHGLTPDQVVAIASNIGGKQALETVQRLLPVLCQDHGLTPDQVVAIASNGGGKQALETVQRLLPVLCQDHGLTPDQVVAIASNIGGKQALETVQRLLPVLCQDHGLTPDQVVAIASNGGGKQALETVQRLLPVLCQDHGLTPDQVVAIASNGGGKQALETVQRLLPVLCQDHGLTPDQVVAIASHDGGKQALETVQRLLPVLCQDHGLTPDQVVAIASHDGGKQALETVQRLLPVLCQDHGLTPDQVVAIASNIGGKQALETVQRLLPVLCQDHGLTPDQVVAIASHDGGKQALETVQRLLPVLCQDHGLTPDQVVAIASNKGGKQALETVQRLLPVLCQDHGLTPDQVVAIASNGGGKQALESIVAQLSRPDPALAALTNDHLVALACLGGRPAMDAVKKGLPHAPELIRRVNRRIGERTSHRVAGSTGGGGGSGTASSKGGRADPAFLYKVVDTEDVVCCSMSYTWTGKGSSSSSRMVSKGEEDNMAIIKEFMRFKVHMEGSVNGHEFEIEGEGEGRPYEGTQTAKLKVTKGGPLPFAWDILSPQFMYGSKAYVKHPADIPDYLKLSFPEGFKWERVMNFEDGGVVTVTQDSSLQDGEFIYKVKLRGTNFPSDGPVMQKKTMGWEASSERMYPEDGALKGEIKQRLKLKDGGHYDAEVKTTYKAKKPVQLPGAYNVNIKLDITSHNEDYTIVEQYERAEGRHSTGGMDELYKKSLGSAHIVMVDAYKPTKSRRPGILYK

SEQ ID NO: 79 - RNA, 4090 nt, synthetic construct
  source 1..4090: mol_type = other RNA
gttttcccagtcacgacgttgtaaaacgacggccagtgaattgtaatacgactcactatagggcgaattaattcgagctcggtacccagcttgcttgttctttttgcagaagctcagaataaacgctcaactttggcagatcaattccccggtgctagcatggatagtgctacccatattaaattctcaaaacgtgatgaggacggcaaagagttagctggtgcaactatggagttgcgtgattcatctggtaaaactattagtacatggatttcagatggacaagtgaaagatttctacctgtatccaggaaaatatacatttgtcgaaaccgcagcaccagacggttatgaggtagcaactgctattacctttacagttaatgagcaaggtcaggttactgtaaatggcaaagcaactaaaggtgacgctcatattggatccaccggtggttccagttctgacaccgaggacgtggtgtgctgcagcatgagctacacctggaccggcaagactacaagtttgtacaaaaaagcaggctccgcggccgcccccttcaccatgcaggtggatctacgcacgctcggctacagtcagcagcagcaagagaagatcaaaccgaaggtgcgttcgacagtggcgcagcaccacgaggcactggtgggccatgggtttacacacgcgcacatcgttgcgctcagccaacacccggcagcgttagggaccgtcgctgtcacgtatcagcacataatcacggcgttgccagaggcgacacacgaagacatcgttggcgtcggcaaacagtggtccggcgcacgcgccctggaggccttgctcacggatgcgggggagttgagaggtccgccgttacagttggacacaggccaacttgtgaagattgcaaaacgtggcggcgtgaccgcaatggaggcagtgcatgcatcgcgcaatgcactgacgggtgcccccctgaacctgaccccggaccaagtggtggctatcgccagcaacggtggcggcaagcaagcgctcgaaacggtgcagcggctgttgccggtgctgtgccaggaccatggcctgaccccggaccaagtggtggctatcgccagcaacaagggcggcaagcaagcgctcgaaacggtgcagcggctgttgccggtgctgtgccaggaccatggcctgactccggaccaagtggtggctatcgccagccacgatggcggcaagcaagcgctcgaaacggtgcagcggctgttgccggtgctgtgccaggaccatggcctgactccggaccaagtggtggctatcgccagccacgatggcggcaagcaagcgctcgaaacggtgcagcggctgttgccggtgctgtgccaggaccatggcctgaccccggaccaagtggtggctatcgccagcaacattggcggcaagcaagcgctcgaaacggtgcagcggctgttgccggtgctgtgccaggaccatggcctgaccccggaccaagtggtggctatcgccagcaacggtggcggcaagcaagcgctcgaaacggtgcagcggctgttgccggtgctgtgccaggaccatggcctgaccccggaccaagtggtggctatcgccagcaacattggcggcaagcaagcgctcgaaacggtgcagcggctgttgccggtgctgtgccaggaccatggcctgaccccggaccaagtggtggctatcgccagcaacggtggcggcaagcaagcgctcgaaacggtgcagcggctgttgccggtgctgtgccaggaccatggcctgaccccggaccaagtggtggctatcgccagcaacggtggcggcaagcaagcgctcgaaacggtgcagcggctgttgccggtgctgtgccaggaccatggcctgactccggaccaagtggtggctatcgccagccacgatggcggcaagcaagcgctcgaaacggtgcagcggctgttgccggtgctgtgccaggaccatggcctgaccccggaccaagtggtggctatcgccagccacgatggcggcaagcaagcgctcgaaacggtgcagcggctgttgccggtgctgtgccaggaccatggcctgaccccggaccaagtggtggctatcgccagcaacattggcggcaagcaagcgctcgaaacggtgcagcggctgttgccggtgctgtgccaggaccatggcctgactccggaccaagtggtggctatcgccagccacgatggcggcaagcaagcgctcgaaacggtgcagcggctgttgccggtgctgtgccaggaccatggcctgaccccggaccaagtggtggctatcgccagcaacaagggcggcaagcaagcgctcgaaacggtgcagcggctgttgccggtgctgtgccaggaccatggcctgaccccggaccaagtggtggctatcgccagcaacggtggcggcaagcaagcgctcgaaagcattgtggcccagctgagccggcctgatccggcgttggccgcgttgaccaacgaccacctcgtcgccttggcctgcctcggcggacgtcctgccatggatgcagtgaaaaagggattgccgcacgcgccggaattgatcagaagagtcaatcgccgtattggcgaacgcacgtcccatcgcgttgcgggatccactggaggcggaggtggctccggcaccgcctcctccaagggtgggcgcgccgacccagctttcttgtacaaagtggttgacactgaggatgtagtatgctgtagcatgagttacacttggacaggcaagggatcaagttcatcctcgagctcaagcttcgaattcatggtgagcaagggcgaggagctgttcaccggggtggtgcccatcctggtcgagctggacggcgacgtaaacgaccacaagttcagcgtccgcggcgagggcgagggcgatgccaccaacggcaagctgaccctgaagttcatctgcaccaccggcaagctgcccgtgccctggcccaccctcgtgaccaccttcggctacggcgtggcctgcttcagccgctaccccgaccacatgaagcagcacgacttcttcaagtccgccatgcccgaaggctacgtccaggagcgcaccatctctttcaaggacgacggtacctacaagacccgcgccgaggtgaagttcgagggcgacaccctggtgaaccgcatcgagctgaagggcatcgacttcaaggaggacggcaacatcctggggcacaagctggagtacaacttcaacagccacaacgtctatatcacggccgacaagcagaagaacggcatcaaggctaacttcaagatccgccacaacgttgaggacggcagcgtgcagctcgccgaccactaccagcagaacacccccatcggcgacggccccgtgctgctgcccgacaaccactacctgagccatcagtccaagctgagcaaagaccccaacgagaagcgcgatcacatggtcctgctggagttcgtgaccgccgccgggattacacatggcatggacgagctgtacaaggtcgacatggatagtgctacccatattaaattctcaaaacgtgatgaggacggcaaagagttagctggtgcaactatggagttgcgtgattcatctggtaaaactattagtacatggatttcagatggacaagtgaaagatttctacctgtatccaggaaaatatacatttgtcgaaaccgcagcaccagacggttatgaggtagcaactgctattacctttacagttaatgagcaaggtcaggttactgtaaatggcaaagcaactaaaggtgacgctcatattggatcctaagcggccgctctagataaatgatagcttgatctggttaccactaaaccagcctcaagaacacccgaatggagtctctaagctacataataccaacttacactttacaaaatgttgtcccccaaaatgtagccattcgtatctgctcctaataaaaagaaagtttcttcacattctaaaaaaaaaaaaaaaaaaaaaaaaaaaaaaaaaaccccccccccccccccctgcaggcgcgccgccggcgatttaaattaat

SEQ ID NO: 80 - protein, 1224 aa, synthetic construct
MDSATHIKFSKRDEDGKELAGATMELRDSSGKTISTWISDGQVKDFYLYPGKYTFVETAAPDGYEVATAITFTVNEQGQVTVNGKATKGDAHIGSTGGSSSDTEDVVCCSMSYTWTGKTTSLYKKAGSAAAPFTMQVDLRTLGYSQQQQEKIKPKVRSTVAQHHEALVGHGFTHAHIVALSQHPAALGTVAVTYQHIITALPEATHEDIVGVGKQWSGARALEALLTDAGELRGPPLQLDTGQLVKIAKRGGVTAMEAVHASRNALTGAPLNLTPDQVVAIASNGGGKQALETVQRLLPVLCQDHGLTPDQVVAIASNKGGKQALETVQRLLPVLCQDHGLTPDQVVAIASHDGGKQALETVQRLLPVLCQDHGLTPDQVVAIASHDGGKQALETVQRLLPVLCQDHGLTPDQVVAIASNIGGKQALETVQRLLPVLCQDHGLTPDQVVAIASNGGGKQALETVQRLLPVLCQDHGLTPDQVVAIASNIGGKQALETVQRLLPVLCQDHGLTPDQVVAIASNGGGKQALETVQRLLPVLCQDHGLTPDQVVAIASNGGGKQALETVQRLLPVLCQDHGLTPDQVVAIASHDGGKQALETVQRLLPVLCQDHGLTPDQVVAIASHDGGKQALETVQRLLPVLCQDHGLTPDQVVAIASNIGGKQALETVQRLLPVLCQDHGLTPDQVVAIASHDGGKQALETVQRLLPVLCQDHGLTPDQVVAIASNKGGKQALETVQRLLPVLCQDHGLTPDQVVAIASNGGGKQALESIVAQLSRPDPALAALTNDHLVALACLGGRPAMDAVKKGLPHAPELIRRVNRRIGERTSHRVAGSTGGGGGSGTASSKGGRADPAFLYKVVDTEDVVCCSMSYTWTGKGSSSSSSSSFEFMVSKGEELFTGVVPILVELDGDVNDHKFSVRGEGEGDATNGKLTLKFICTTGKLPVPWPTLVTTFGYGVACFSRYPDHMKQHDFFKSAMPEGYVQERTISFKDDGTYKTRAEVKFEGDTLVNRIELKGIDFKEDGNILGHKLEYNFNSHNVYITADKQKNGIKANFKIRHNVEDGSVQLADHYQQNTPIGDGPVLLPDNHYLSHQSKLSKDPNEKRDHMVLLEFVTAAGITHGMDELYKVDMDSATHIKFSKRDEDGKELAGATMELRDSSGKTISTWISDGQVKDFYLYPGKYTFVETAAPDGYEVATAITFTVNEQGQVTVNGKATKGDAHIGS